European Patent Specification EP 3 443 006 B1, published August 2, 2023. Title: TRISPECIFIC AND/OR TRIVALENT BINDING PROTEINS. Applicant: YANG, Zhi-yong NABEL, Gary J. WU, Lan SEUNG, Edward WEI, Ronnie BENINGA, Jochen RAO, Ercole LEUSCHNER, Wulf Dirk BEIL, Christian LANGE, Christian CORVEY, Carsten. Application Not Yet Assigned. The sequence listing filed with the application follows.

SEQUENCE LISTING (179 sequences)

SEQ ID NO: 1 - protein, 447 aa, Artificial Sequence
  Synthetic Construct
EVQLVESGGGLVQPGGSLRLSCAASGFNIKDTYIHWVRQAPGKGLEWVARIYPTNGYTRYADSVKGRFTISADTSKNTAYLQMNSLRAEDTAVYYCSRWGGDGFYAMDYWGQGTLVTVSSASTKGPSVFPLAPCSRSTSESTAALGCLVKDYFPEPVTVSWNSGALTSGVHTFPAVLQSSGLYSLSSVVTVPSSSLGTKTYTCNVDHKPSNTKVDKRVESKYGPPCPPCPAPEFLGGPSVFLFPPKPKDTLMISRTPEVTCVVVDVSQEDPEVQFNWYVDGVEVHNAKTKPREEQFNSTYRVVSVLTVLHQDWLNGKEYKCKVSNKGLPSSIEKTISKAKGQPREPQVYTLPPCQEEMTKNQVSLWCLVKGFYPSDIAVEWESNGQPENNYKTTPPVLDSDGSFFLYSKLTVDKSRWQEGNVFSCSVMHEALHNHYTQKSLSLSLGK

SEQ ID NO: 2 - protein, 214 aa, Artificial Sequence
  Synthetic Construct
DIQMTQSPSSLSASVGDRVTITCRASQDVNTAVAWYQQKPGKAPKLLIYSASFLYSGVPSRFSGSRSGTDFTLTISSLQPEDFATYYCQQHYTTPPTFGQGTKVEIKRTVAAPSVFIFPPSDEQLKSGTASVVCLLNNFYPREAKVQWKVDNALQSGNSQESVTEQDSKDSTYSLSSTLTLSKADYEKHKVYACEVTHQGLSSPVTKSFNRGEC

SEQ ID NO: 3 - protein, 571 aa, Artificial Sequence
  Synthetic Construct
QVQLVQSGAEVVKPGASVKVSCKASGYTFTSYYIHWVRQAPGQGLEWIGSIYPGNVNTNYAQKFQGRATLTVDTSISTAYMELSRLRSDDTAVYYCTRSHYGLDWNFDVWGKGTTVTVSSSQVQLVESGGGVVQPGRSLRLSCAASGFTFTKAWMHWVRQAPGKQLEWVAQIKDKSNSYATYYADSVKGRFTISRDDSKNTLYLQMNSLRAEDTAVYYCRGVYYALSPFDYWGQGTLVTVSSRTASTKGPSVFPLAPCSRSTSESTAALGCLVKDYFPEPVTVSWNSGALTSGVHTFPAVLQSSGLYSLSSVVTVPSSSLGTKTYTCNVDHKPSNTKVDKRVESKYGPPCPPCPAPEFLGGPSVFLFPPKPKDTLMISRTPEVTCVVVDVSQEDPEVQFNWYVDGVEVHNAKTKPREEQFNSTYRVVSVLTVLHQDWLNGKEYKCKVSNKGLPSSIEKTISKAKGQPREPQVCTLPPSQEEMTKNQVSLSCAVKGFYPSDIAVEWESNGQPENNYKTTPPVLDSDGSFFLVSKLTVDKSRWQEGNVFSCSVMHEALHNHYTQKSLSLSLGK

SEQ ID NO: 4 - protein, 338 aa, Artificial Sequence
  Synthetic Construct
DIVMTQTPLSLSVTPGQPASISCKSSQSLVHNNANTYLSWYLQKPGQSPQSLIYKVSNRFSGVPDRFSGSGSGTDFTLKISRVEAEDVGVYYCGQGTQYPFTFGSGTKVEIKGQPKAAPDIQMTQSPSSLSASVGDRVTITCQASQNIYVWLNWYQQKPGKAPKLLIYKASNLHTGVPSRFSGSGSGTDFTLTISSLQPEDIATYYCQQGQTYPYTFGQGTKLEIKTKGPSRTVAAPSVFIFPPSDEQLKSGTASVVCLLNNFYPREAKVQWKVDNALQSGNSQESVTEQDSKDSTYSLSSTLTLSKADYEKHKVYACEVTHQGLSSPVTKSFNRGEC

SEQ ID NO: 5 - DNA, 1341 bp, Artificial Sequence
  Synthetic Construct
gaagtgcagctggtggaatctggcggcggactggtgcagcctggcggatctctgagactgagctgtgccgccagcggcttcaacatcaaggacacctacatccactgggtgcgccaggcccctggcaagggactggaatgggtggccagaatctaccccaccaacggctacaccagatacgccgacagcgtgaagggccggttcaccatcagcgccgacaccagcaagaacaccgcctacctgcagatgaacagcctgcgggccgaggacaccgccgtgtactactgtagtagatggggaggcgacggcttctacgccatggactattggggccagggcaccctcgtgaccgtgtctagtgcgtcgaccaagggcccatcggtgttccctctggccccttgcagcagaagcaccagcgaatctacagccgccctgggctgcctcgtgaaggactactttcccgagcccgtgaccgtgtcctggaactctggcgctctgacaagcggcgtgcacacctttccagccgtgctccagagcagcggcctgtactctctgagcagcgtcgtgacagtgcccagcagcagcctgggcaccaagacctacacctgtaacgtggaccacaagcccagcaacaccaaggtggacaagcgggtggaatctaagtacggccctccctgccctccttgcccagcccctgaatttctgggcggaccctccgtgttcctgttccccccaaagcccaaggacaccctgatgatcagccggacccccgaagtgacctgcgtggtggtggatgtgtcccaggaagatcccgaggtgcagttcaattggtacgtggacggcgtggaagtgcacaacgccaagaccaagcccagagaggaacagttcaacagcacctaccgggtggtgtccgtgctgaccgtgctgcaccaggactggctgaacggcaaagagtacaagtgcaaggtgtccaacaagggcctgcccagctccatcgagaaaaccatcagcaaggccaagggccagccccgcgagcctcaagtgtataccctgcccccttgccaggaagagatgaccaagaaccaggtgtccctgtggtgtctcgtgaaaggcttctaccccagcgacattgccgtggaatgggagagcaacggccagcccgagaacaactacaagaccaccccccctgtgctggacagcgacggctcattcttcctgtactccaagctgaccgtggacaagagccggtggcaggaaggcaacgtgttcagctgctccgtgatgcacgaggccctgcacaaccactacacccagaagtccctgtctctgtccctgggcaag

SEQ ID NO: 6 - DNA, 642 bp, Artificial Sequence
  Synthetic Construct
gacatccagatgacccagagccccagcagcctgtctgccagcgtgggcgacagagtgaccatcacctgtagagccagccaggacgtgaacaccgccgtggcctggtatcagcagaagcctggcaaggcccccaagctgctgatctacagcgccagcttcctgtacagcggcgtgcccagcagattcagcggaagcagaagcggcaccgacttcaccctgaccatcagctccctgcagcccgaggacttcgccacctactactgccagcagcactacaccaccccccccacatttggccagggcaccaaggtggaaatcaagcgtacggtggccgctcccagcgtgttcatcttcccacctagcgacgagcagctgaagtccggcacagcctctgtcgtgtgcctgctgaacaacttctacccccgcgaggccaaagtgcagtggaaggtggacaacgccctgcagagcggcaacagccaggaaagcgtgaccgagcaggacagcaaggactccacctacagcctgagcagcaccctgacactgagcaaggccgactacgagaagcacaaggtgtacgcctgcgaagtgacccaccagggcctgtctagccccgtgaccaagagcttcaaccggggcgagtgt

SEQ ID NO: 7 - DNA, 1713 bp, Artificial Sequence
  Synthetic Construct
caggtgcagctggtgcagtctggcgccgaggtcgtgaaacctggcgcctctgtgaaggtgtcctgcaaggccagcggctacacctttaccagctactacatccactgggtgcgccaggcccctggacagggactggaatggatcggcagcatctaccccggcaacgtgaacaccaactacgcccagaagttccagggcagagccaccctgaccgtggacaccagcatcagcaccgcctacatggaactgagccggctgagaagcgacgacaccgccgtgtactactgcacccggtcccactacggcctggattggaacttcgacgtgtggggcaagggcaccaccgtgacagtgtctagcagccaggtgcagctggtggaatctggcggcggagtggtgcagcctggcagaagcctgagactgagctgtgccgccagcggcttcaccttcaccaaggcctggatgcactgggtgcgccaggcccctggaaagcagctggaatgggtggcccagatcaaggacaagagcaacagctacgccacctactacgccgacagcgtgaagggccggttcaccatcagccgggacgacagcaagaacaccctgtacctgcagatgaacagcctgcgggccgaggacaccgccgtgtactactgtcggggcgtgtactatgccctgagccccttcgattactggggccagggaaccctcgtgaccgtgtctagtcggaccgccagcacaaagggcccatcggtgttccctctggccccttgcagcagaagcaccagcgaatctacagccgccctgggctgcctcgtgaaggactactttcccgagcccgtgaccgtgtcctggaactctggcgctctgacaagcggcgtgcacacctttccagccgtgctccagagcagcggcctgtactctctgagcagcgtcgtgacagtgcccagcagcagcctgggcaccaagacctacacctgtaacgtggaccacaagcccagcaacaccaaggtggacaagcgggtggaatctaagtacggccctccctgccctccttgcccagcccctgaatttctgggcggaccctccgtgttcctgttccccccaaagcccaaggacaccctgatgatcagccggacccccgaagtgacctgcgtggtggtggatgtgtcccaggaagatcccgaggtgcagttcaattggtacgtggacggcgtggaagtgcacaacgccaagaccaagcccagagaggaacagttcaacagcacctaccgggtggtgtccgtgctgaccgtgctgcaccaggactggctgaacggcaaagagtacaagtgcaaggtgtccaacaagggcctgcccagctccatcgagaaaaccatcagcaaggccaagggccagccccgcgagcctcaagtgtgtaccctgccccctagccaggaagagatgaccaagaaccaggtgtccctgagctgtgccgtgaaaggcttctaccccagcgacattgccgtggaatgggagagcaacggccagcccgagaacaactacaagaccaccccccctgtgctggacagcgacggctcattcttcctggtgtccaagctgaccgtggacaagagccggtggcaggaaggcaacgtgttcagctgctccgtgatgcacgaggccctgcacaaccactacacccagaagtccctgtctctgtccctgggcaag

SEQ ID NO: 8 - DNA, 1014 bp, Artificial Sequence
  Synthetic Construct
gacatcgtgatgacccagacccccctgagcctgagcgtgacacctggacagcctgccagcatcagctgcaagagcagccagagcctggtgcacaacaacgccaacacctacctgagctggtatctgcagaagcccggccagagcccccagtccctgatctacaaggtgtccaacagattcagcggcgtgcccgacagattctccggcagcggctctggcaccgacttcaccctgaagatcagccgggtggaagccgaggacgtgggcgtgtactattgtggccagggcacccagtaccccttcacctttggcagcggcaccaaggtggaaatcaagggccagcccaaggccgcccccgacatccagatgacccagagccccagcagcctgtctgccagcgtgggcgacagagtgaccatcacctgtcaggccagccagaacatctacgtgtggctgaactggtatcagcagaagcccggcaaggcccccaagctgctgatctacaaggccagcaacctgcacaccggcgtgcccagcagattttctggcagcggctccggcaccgacttcaccctgacaatcagctccctgcagcccgaggacattgccacctactactgccagcagggccagacctacccctacacctttggccagggcaccaagctggaaatcaagaccaagggccccagccgtacggtggccgctcccagcgtgttcatcttcccacctagcgacgagcagctgaagtccggcacagcctctgtcgtgtgcctgctgaacaacttctacccccgcgaggccaaagtgcagtggaaggtggacaacgccctgcagagcggcaacagccaggaaagcgtgaccgagcaggacagcaaggactccacctacagcctgagcagcaccctgacactgagcaaggccgactacgagaagcacaaggtgtacgcctgcgaagtgacccaccagggcctgtctagccccgtgaccaagagcttcaaccggggcgagtgt

SEQ ID NO: 9 - protein, 571 aa, Artificial Sequence
  Synthetic Construct
QVQLQESGPGLVKPSQTLSLTCTVSGFSLSDYGVHWVRQPPGKGLEWLGVIWAGGGTNYNPSLKSRKTISKDTSKNQVSLKLSSVTAADTAVYYCARDKGYSYYYSMDYWGQGTTVTVSSSQVQLVESGGGVVQPGRSLRLSCAASGFTFTKAWMHWVRQAPGKQLEWVAQIKDKSNSYATYYADSVKGRFTISRDDSKNTLYLQMNSLRAEDTAVYYCRGVYYALSPFDYWGQGTLVTVSSRTASTKGPSVFPLAPCSRSTSESTAALGCLVKDYFPEPVTVSWNSGALTSGVHTFPAVLQSSGLYSLSSVVTVPSSSLGTKTYTCNVDHKPSNTKVDKRVESKYGPPCPPCPAPEFLGGPSVFLFPPKPKDTLMISRTPEVTCVVVDVSQEDPEVQFNWYVDGVEVHNAKTKPREEQFNSTYRVVSVLTVLHQDWLNGKEYKCKVSNKGLPSSIEKTISKAKGQPREPQVCTLPPSQEEMTKNQVSLSCAVKGFYPSDIAVEWESNGQPENNYKTTPPVLDSDGSFFLVSKLTVDKSRWQEGNVFSCSVMHEALHNHYTQKSLSLSLGK

SEQ ID NO: 10 - protein, 342 aa, Artificial Sequence
  Synthetic Construct
DIVMTQTPLSLSVTPGQPASISCKSSQSLVHNNANTYLSWYLQKPGQSPQSLIYKVSNRFSGVPDRFSGSGSGTDFTLKISRVEAEDVGVYYCGQGTQYPFTFGSGTKVEIKGQPKAAPDIVLTQSPASLAVSPGQRATITCRASESVEYYVTSLMQWYQQKPGQPPKLLIFAASNVESGVPARFSGSGSGTDFTLTINPVEANDVANYYCQQSRKVPYTFGQGTKLEIKTKGPSRTVAAPSVFIFPPSDEQLKSGTASVVCLLNNFYPREAKVQWKVDNALQSGNSQESVTEQDSKDSTYSLSSTLTLSKADYEKHKVYACEVTHQGLSSPVTKSFNRGEC

SEQ ID NO: 11 - DNA, 1713 bp, Artificial Sequence
  Synthetic Construct
caggtgcagctgcaggaatctggccctggcctcgtgaagcctagccagaccctgagcctgacctgtaccgtgtccggcttcagcctgagcgactacggcgtgcactgggtgcgccagccacctggaaaaggcctggaatggctgggcgtgatctgggctggcggaggcaccaactacaaccccagcctgaagtccagaaagaccatcagcaaggacaccagcaagaaccaggtgtccctgaagctgagcagcgtgacagccgccgataccgccgtgtactactgcgccagagacaagggctacagctactactacagcatggactactggggccagggcaccaccgtgaccgtgtcatcctctcaggtgcagctggtggaatctggcggcggagtggtgcagcctggcagaagcctgagactgagctgtgccgccagcggcttcaccttcaccaaggcctggatgcactgggtgcgccaggcccctggaaagcagctggaatgggtggcccagatcaaggacaagagcaacagctacgccacctactacgccgacagcgtgaagggccggttcaccatcagccgggacgacagcaagaacaccctgtacctgcagatgaacagcctgcgggccgaggacaccgccgtgtactactgtcggggcgtgtactatgccctgagccccttcgattactggggccagggaaccctcgtgaccgtgtctagtcggaccgcttcgaccaagggcccatcggtgttccctctggccccttgcagcagaagcaccagcgaatctacagccgccctgggctgcctcgtgaaggactactttcccgagcccgtgaccgtgtcctggaactctggcgctctgacaagcggcgtgcacacctttccagccgtgctccagagcagcggcctgtactctctgagcagcgtcgtgacagtgcccagcagcagcctgggcaccaagacctacacctgtaacgtggaccacaagcccagcaacaccaaggtggacaagcgggtggaatctaagtacggccctccctgccctccttgcccagcccctgaatttctgggcggaccctccgtgttcctgttccccccaaagcccaaggacaccctgatgatcagccggacccccgaagtgacctgcgtggtggtggatgtgtcccaggaagatcccgaggtgcagttcaattggtacgtggacggcgtggaagtgcacaacgccaagaccaagcccagagaggaacagttcaacagcacctaccgggtggtgtccgtgctgaccgtgctgcaccaggactggctgaacggcaaagagtacaagtgcaaggtgtccaacaagggcctgcccagctccatcgagaaaaccatcagcaaggccaagggccagccccgcgagcctcaagtgtgtaccctgccccctagccaggaagagatgaccaagaaccaggtgtccctgagctgtgccgtgaaaggcttctaccccagcgacattgccgtggaatgggagagcaacggccagcccgagaacaactacaagaccaccccccctgtgctggacagcgacggctcattcttcctggtgtccaagctgaccgtggacaagagccggtggcaggaaggcaacgtgttcagctgctccgtgatgcacgaggccctgcacaaccactacacccagaagtccctgtctctgtccctgggcaag

SEQ ID NO: 12 - DNA, 1026 bp, Artificial Sequence
  Synthetic Construct
gacatcgtgatgacccagacccccctgagcctgagcgtgacacctggacagcctgccagcatcagctgcaagagcagccagagcctggtgcacaacaacgccaacacctacctgagctggtatctgcagaagcccggccagagcccccagtccctgatctacaaggtgtccaacagattcagcggcgtgcccgacagattctccggcagcggctctggcaccgacttcaccctgaagatcagccgggtggaagccgaggacgtgggcgtgtactattgtggccagggcacccagtaccccttcacctttggcagcggcaccaaggtggaaatcaagggccagcccaaggccgcccccgacatcgtgctgacacagagccctgctagcctggccgtgtctcctggacagagggccaccatcacctgtagagccagcgagagcgtggaatattacgtgaccagcctgatgcagtggtatcagcagaagcccggccagccccccaagctgctgattttcgccgccagcaacgtggaaagcggcgtgccagccagattttccggcagcggctctggcaccgacttcaccctgaccatcaaccccgtggaagccaacgacgtggccaactactactgccagcagagccggaaggtgccctacacctttggccagggcaccaagctggaaatcaagaccaagggccccagccgtacggtggccgctcccagcgtgttcatcttcccacctagcgacgagcagctgaagtccggcacagcctctgtcgtgtgcctgctgaacaacttctacccccgcgaggccaaagtgcagtggaaggtggacaacgccctgcagagcggcaacagccaggaaagcgtgaccgagcaggacagcaaggactccacctacagcctgagcagcaccctgacactgagcaaggccgactacgagaagcacaaggtgtacgcctgcgaagtgacccaccagggcctgtctagccccgtgaccaagagcttcaaccggggcgagtgt

SEQ ID NO: 13 - protein, 451 aa, Artificial Sequence
  Synthetic Construct
QVQLVQSGAEVKKPGSSVKVSCKASGYAFSSYWMNWVRQAPGQGLEWIGQIWPGDGDTNYNQKFKGRATLTADESTSTAYMELSSLRSEDTAVYYCARRETTTVGRYYYAMDYWGQGTTVTVSSASTKGPSVFPLAPCSRSTSESTAALGCLVKDYFPEPVTVSWNSGALTSGVHTFPAVLQSSGLYSLSSVVTVPSSSLGTKTYTCNVDHKPSNTKVDKRVESKYGPPCPPCPAPEFLGGPSVFLFPPKPKDTLMISRTPEVTCVVVDVSQEDPEVQFNWYVDGVEVHNAKTKPREEQFNSTYRVVSVLTVLHQDWLNGKEYKCKVSNKGLPSSIEKTISKAKGQPREPQVYTLPPCQEEMTKNQVSLWCLVKGFYPSDIAVEWESNGQPENNYKTTPPVLDSDGSFFLYSKLTVDKSRWQEGNVFSCSVMHEALHNHYTQKSLSLSLGK

SEQ ID NO: 14 - protein, 218 aa, Artificial Sequence
  Synthetic Construct
DLVLTQSPASLAVSPGQRATITCKASQSVDYDGDSYLNWYQQKPGQPPKLLIYDASNLVSGVPARFSGSGSGTDFTLTINPVEANDTANYYCQQSTEDPWTFGQGTKLEIKRTVAAPSVFIFPPSDEQLKSGTASVVCLLNNFYPREAKVQWKVDNALQSGNSQESVTEQDSKDSTYSLSSTLTLSKADYEKHKVYACEVTHQGLSSPVTKSFNRGEC

SEQ ID NO: 15 - DNA, 1353 bp, Artificial Sequence
  Synthetic Construct
caggtgcagctggtgcagagcggcgccgaagtgaagaagcctggcagcagcgtgaaggtgagctgcaaggccagcggctatgccttcagcagctactggatgaactgggtgaggcaggcacctggccagggcctggagtggataggccaaatatggcctggcgatggcgacaccaactacaaccagaagttcaagggcagagcgaccttgaccgccgacgagagcaccagcaccgcgtacatggagctgagcagcctgaggagcgaggacaccgccgtgtactattgcgccagaagggagaccaccaccgtgggcaggtactactacgccatggactactggggccagggaaccaccgtgaccgtgagcagcgcctcgaccaagggcccatcggtgttccctctggccccttgcagcagaagcaccagcgaatctacagccgccctgggctgcctcgtgaaggactactttcccgagcccgtgaccgtgtcctggaactctggcgctctgacaagcggcgtgcacacctttccagccgtgctccagagcagcggcctgtactctctgagcagcgtcgtgacagtgcccagcagcagcctgggcaccaagacctacacctgtaacgtggaccacaagcccagcaacaccaaggtggacaagcgggtggaatctaagtacggccctccctgccctccttgcccagcccctgaatttctgggcggaccctccgtgttcctgttccccccaaagcccaaggacaccctgatgatcagccggacccccgaagtgacctgcgtggtggtggatgtgtcccaggaagatcccgaggtgcagttcaattggtacgtggacggcgtggaagtgcacaacgccaagaccaagcccagagaggaacagttcaacagcacctaccgggtggtgtccgtgctgaccgtgctgcaccaggactggctgaacggcaaagagtacaagtgcaaggtgtccaacaagggcctgcccagctccatcgagaaaaccatcagcaaggccaagggccagccccgcgagcctcaagtgtataccctgcccccttgccaggaagagatgaccaagaaccaggtgtccctgtggtgtctcgtgaaaggcttctaccccagcgacattgccgtggaatgggagagcaacggccagcccgagaacaactacaagaccaccccccctgtgctggacagcgacggctcattcttcctgtactccaagctgaccgtggacaagagccggtggcaggaaggcaacgtgttcagctgctccgtgatgcacgaggccctgcacaaccactacacccagaagtccctgtctctgtccctgggcaag

SEQ ID NO: 16 - DNA, 654 bp, Artificial Sequence
  Synthetic Construct
gacctcgtgctgacccagagccctgcgagcctggctgtgagccctggccagagagccaccatcacctgcaaagccagccagagcgtggactacgacggcgacagctacctcaactggtaccagcagaagcctggccagccccccaagctgctgatttacgatgccagcaacctggtgagcggcgtgcctgctagattcagcggctccggcagcggcaccgacttcaccctgaccatcaaccccgtggaggccaacgacaccgccaactactactgccagcagagcacggaggacccctggaccttcggccagggcacaaagctggagatcaagcgtacggtggccgctcccagcgtgttcatcttcccacctagcgacgagcagctgaagtccggcacagcctctgtcgtgtgcctgctgaacaacttctacccccgcgaggccaaagtgcagtggaaggtggacaacgccctgcagagcggcaacagccaggaaagcgtgaccgagcaggacagcaaggactccacctacagcctgagcagcaccctgacactgagcaaggccgactacgagaagcacaaggtgtacgcctgcgaagtgacccaccagggcctgtctagccccgtgaccaagagcttcaaccggggcgagtgt

SEQ ID NO: 17 - protein, 447 aa, Artificial Sequence
  Synthetic Construct
QVQLVQSGAEVAKPGTSVKLSCKASGYTFTDYWMQWVKQRPGQGLEWIGTIYPGDGDTGYAQKFQGKATLTADKSSKTVYMHLSSLASEDSAVYYCARGDYYGSNSLDYWGQGTSVTVSSASTKGPSVFPLAPCSRSTSESTAALGCLVKDYFPEPVTVSWNSGALTSGVHTFPAVLQSSGLYSLSSVVTVPSSSLGTKTYTCNVDHKPSNTKVDKRVESKYGPPCPPCPAPEFLGGPSVFLFPPKPKDTLMISRTPEVTCVVVDVSQEDPEVQFNWYVDGVEVHNAKTKPREEQFNSTYRVVSVLTVLHQDWLNGKEYKCKVSNKGLPSSIEKTISKAKGQPREPQVYTLPPCQEEMTKNQVSLWCLVKGFYPSDIAVEWESNGQPENNYKTTPPVLDSDGSFFLYSKLTVDKSRWQEGNVFSCSVMHEALHNHYTQKSLSLSLGK

SEQ ID NO: 18 - protein, 214 aa, Artificial Sequence
  Synthetic Construct
DIVMTQSHLSMSTSLGDPVSITCKASQDVSTVVAWYQQKPGQSPRRLIYSASYRYIGVPDRFTGSGAGTDFTFTISSVQAEDLAVYYCQQHYSPPYTFGGGTKLEIKRTVAAPSVFIFPPSDEQLKSGTASVVCLLNNFYPREAKVQWKVDNALQSGNSQESVTEQDSKDSTYSLSSTLTLSKADYEKHKVYACEVTHQGLSSPVTKSFNRGEC

SEQ ID NO: 19 - DNA, 1341 bp, Artificial Sequence
  Synthetic Construct
caggtgcagctggtgcagtctggcgccgaagtggccaagcctggcacaagcgtgaagctgagctgcaaggccagcggctacaccttcaccgactactggatgcagtgggtcaagcagaggccaggccagggcctggaatggatcggcacaatctatcccggcgacggcgataccggctacgcccagaagtttcagggcaaggccaccctgaccgccgacaagagcagcaagaccgtgtacatgcacctgagcagcctggccagcgaggacagcgccgtgtactattgcgccagaggcgactactacggcagcaacagcctggactattggggccagggcaccagcgtgacagtgtctagtgcgtcgaccaagggcccatcggtgttccctctggccccttgcagcagaagcaccagcgaatctacagccgccctgggctgcctcgtgaaggactactttcccgagcccgtgaccgtgtcctggaactctggcgctctgacaagcggcgtgcacacctttccagccgtgctccagagcagcggcctgtactctctgagcagcgtcgtgacagtgcccagcagcagcctgggcaccaagacctacacctgtaacgtggaccacaagcccagcaacaccaaggtggacaagcgggtggaatctaagtacggccctccctgccctccttgcccagcccctgaatttctgggcggaccctccgtgttcctgttccccccaaagcccaaggacaccctgatgatcagccggacccccgaagtgacctgcgtggtggtggatgtgtcccaggaagatcccgaggtgcagttcaattggtacgtggacggcgtggaagtgcacaacgccaagaccaagcccagagaggaacagttcaacagcacctaccgggtggtgtccgtgctgaccgtgctgcaccaggactggctgaacggcaaagagtacaagtgcaaggtgtccaacaagggcctgcccagctccatcgagaaaaccatcagcaaggccaagggccagccccgcgagcctcaagtgtataccctgcccccttgccaggaagagatgaccaagaaccaggtgtccctgtggtgtctcgtgaaaggcttctaccccagcgacattgccgtggaatgggagagcaacggccagcccgagaacaactacaagaccaccccccctgtgctggacagcgacggctcattcttcctgtactccaagctgaccgtggacaagagccggtggcaggaaggcaacgtgttcagctgctccgtgatgcacgaggccctgcacaaccactacacccagaagtccctgtctctgtccctgggcaag

SEQ ID NO: 20 - DNA, 642 bp, Artificial Sequence
  Synthetic Construct
gacatcgtgatgacccagagccacctgagcatgagcaccagcctgggcgaccccgtgtccatcacctgtaaagccagccaggacgtgtccaccgtggtggcctggtatcagcagaagcctggccagagccccagacggctgatctacagcgccagctatcggtacatcggcgtgcccgacagattcaccggaagcggagccggcaccgacttcaccttcaccatcagctctgtgcaggccgaggacctggccgtgtactactgccagcagcactacagccccccctacacctttggcggaggcaccaagctggaaatcaagcgtacggtggccgctcccagcgtgttcatcttcccacctagcgacgagcagctgaagtccggcacagcctctgtcgtgtgcctgctgaacaacttctacccccgcgaggccaaagtgcagtggaaggtggacaacgccctgcagagcggcaacagccaggaaagcgtgaccgagcaggacagcaaggactccacctacagcctgagcagcaccctgacactgagcaaggccgactacgagaagcacaaggtgtacgcctgcgaagtgacccaccagggcctgtctagccccgtgaccaagagcttcaaccggggcgagtgt

SEQ ID NO: 21 - protein, 445 aa, Artificial Sequence
  Synthetic Construct
QVQLVQSGAEVKKPGSSVKVSCKASGYIFTNYNIHWVKKSPGQGLEWIGAIYPGNGDAPYSQKFQGKATLTADTSTSTTYMELSSLRSEDTAVYYCVRANWDVAFAYWGQGTLVTVSSASTKGPSVFPLAPCSRSTSESTAALGCLVKDYFPEPVTVSWNSGALTSGVHTFPAVLQSSGLYSLSSVVTVPSSSLGTKTYTCNVDHKPSNTKVDKRVESKYGPPCPPCPAPEFLGGPSVFLFPPKPKDTLMISRTPEVTCVVVDVSQEDPEVQFNWYVDGVEVHNAKTKPREEQFNSTYRVVSVLTVLHQDWLNGKEYKCKVSNKGLPSSIEKTISKAKGQPREPQVYTLPPCQEEMTKNQVSLWCLVKGFYPSDIAVEWESNGQPENNYKTTPPVLDSDGSFFLYSKLTVDKSRWQEGNVFSCSVMHEALHNHYTQKSLSLSLGK

SEQ ID NO: 22 - protein, 213 aa, Artificial Sequence
  Synthetic Construct
DIQMTQSPSSLSASVGDRVTITCKASQDIDRYMAWYQDKPGKAPRLLIHDTSTLQSGVPSRFSGSGSGRDYTLTISNLEPEDFATYYCLQYDNLWTFGGGTKVEIKRTVAAPSVFIFPPSDEQLKSGTASVVCLLNNFYPREAKVQWKVDNALQSGNSQESVTEQDSKDSTYSLSSTLTLSKADYEKHKVYACEVTHQGLSSPVTKSFNRGEC

SEQ ID NO: 23 - DNA, 1335 bp, Artificial Sequence
  Synthetic Construct
caggtgcagctggtgcagtctggcgccgaagtgaagaaacccggcagcagcgtgaaggtgtcctgcaaggccagcggctacatcttcaccaactacaacatccactgggtcaagaagtccccaggccagggcctggaatggatcggcgccatctatcccggaaacggcgacgccccttacagccagaagttccagggcaaggccaccctgaccgccgataccagcacctccaccacctacatggaactgagcagcctgcggagcgaggacaccgccgtgtactattgcgtgcgggccaactgggatgtggccttcgcctattggggccagggcacactcgtgaccgtgtcctctgcgtcgaccaagggcccatcggtgttccctctggccccttgcagcagaagcaccagcgaatctacagccgccctgggctgcctcgtgaaggactactttcccgagcccgtgaccgtgtcctggaactctggcgctctgacaagcggcgtgcacacctttccagccgtgctccagagcagcggcctgtactctctgagcagcgtcgtgacagtgcccagcagcagcctgggcaccaagacctacacctgtaacgtggaccacaagcccagcaacaccaaggtggacaagcgggtggaatctaagtacggccctccctgccctccttgcccagcccctgaatttctgggcggaccctccgtgttcctgttccccccaaagcccaaggacaccctgatgatcagccggacccccgaagtgacctgcgtggtggtggatgtgtcccaggaagatcccgaggtgcagttcaattggtacgtggacggcgtggaagtgcacaacgccaagaccaagcccagagaggaacagttcaacagcacctaccgggtggtgtccgtgctgaccgtgctgcaccaggactggctgaacggcaaagagtacaagtgcaaggtgtccaacaagggcctgcccagctccatcgagaaaaccatcagcaaggccaagggccagccccgcgagcctcaagtgtataccctgcccccttgccaggaagagatgaccaagaaccaggtgtccctgtggtgtctcgtgaaaggcttctaccccagcgacattgccgtggaatgggagagcaacggccagcccgagaacaactacaagaccaccccccctgtgctggacagcgacggctcattcttcctgtactccaagctgaccgtggacaagagccggtggcaggaaggcaacgtgttcagctgctccgtgatgcacgaggccctgcacaaccactacacccagaagtccctgtctctgtccctgggcaag

SEQ ID NO: 24 - DNA, 639 bp, Artificial Sequence
  Synthetic Construct
gacatccagatgacccagagccccagcagcctgtctgccagcgtgggcgacagagtgaccatcacatgcaaggccagccaggacatcgatcggtacatggcctggtatcaggacaagcccggcaaggcccccagactgctgatccacgataccagcacactgcagagcggcgtgcccagcagattttccggctctggcagcggcagagactacaccctgaccatcagcaacctggaacccgaggacttcgccacctactactgcctgcagtacgacaacctgtggaccttcggcggaggcaccaaggtggaaatcaagcgtacggtggccgctcccagcgtgttcatcttcccacctagcgacgagcagctgaagtccggcacagcctctgtcgtgtgcctgctgaacaacttctacccccgcgaggccaaagtgcagtggaaggtggacaacgccctgcagagcggcaacagccaggaaagcgtgaccgagcaggacagcaaggactccacctacagcctgagcagcaccctgacactgagcaaggccgactacgagaagcacaaggtgtacgcctgcgaagtgacccaccagggcctgtctagccccgtgaccaagagcttcaaccggggcgagtgt

SEQ ID NO: 25 - protein, 8 aa, Artificial Sequence
  Synthetic Construct
GFNIKDTY

SEQ ID NO: 26 - protein, 8 aa, Artificial Sequence
  Synthetic Construct
IYPTNGYT

SEQ ID NO: 27 - protein, 13 aa, Artificial Sequence
  Synthetic Construct
SRWGGDGFYAMDY

SEQ ID NO: 28 - protein, 8 aa, Artificial Sequence
  Synthetic Construct
GYTFTSYY

SEQ ID NO: 29 - protein, 8 aa, Artificial Sequence
  Synthetic Construct
IYPGNVNT

SEQ ID NO: 30 - protein, 13 aa, Artificial Sequence
  Synthetic Construct
TRSHYGLDWNFDV

SEQ ID NO: 31 - protein, 8 aa, Artificial Sequence
  Synthetic Construct
GFSLSDYG

SEQ ID NO: 32 - protein, 7 aa, Artificial Sequence
  Synthetic Construct
IWAGGGT

SEQ ID NO: 33 - protein, 13 aa, Artificial Sequence
  Synthetic Construct
ARDKGYSYYYSMD

SEQ ID NO: 34 - protein, 8 aa, Artificial Sequence
  Synthetic Construct
GFTFTKAW

SEQ ID NO: 35 - protein, 7 aa, Artificial Sequence
  Synthetic Construct
IKDKSNS

SEQ ID NO: 36 - protein, 12 aa, Artificial Sequence
  Synthetic Construct
RGVYYALSPFDY

SEQ ID NO: 37 - protein, 8 aa, Artificial Sequence
  Synthetic Construct
GYAFSSYW

SEQ ID NO: 38 - protein, 8 aa, Artificial Sequence
  Synthetic Construct
IWPGDGDT

SEQ ID NO: 39 - protein, 16 aa, Artificial Sequence
  Synthetic Construct
ARRETTTVGRYYYAMD

SEQ ID NO: 40 - protein, 8 aa, Artificial Sequence
  Synthetic Construct
GYTFTDYW

SEQ ID NO: 41 - protein, 8 aa, Artificial Sequence
  Synthetic Construct
IYPGDGDT

SEQ ID NO: 42 - protein, 13 aa, Artificial Sequence
  Synthetic Construct
ARGDYYGSNSLDY

SEQ ID NO: 43 - protein, 6 aa, Artificial Sequence
  Synthetic Construct
QDVNTA

SEQ ID NO: 44 - protein, 3 aa, Artificial Sequence
  Synthetic Construct
SAS

SEQ ID NO: 45 - protein, 9 aa, Artificial Sequence
  Synthetic Construct
QQHYTTPPT

SEQ ID NO: 46 - protein, 6 aa, Artificial Sequence
  Synthetic Construct
QNIYVW

SEQ ID NO: 47 - protein, 3 aa, Artificial Sequence
  Synthetic Construct
KAS

SEQ ID NO: 48 - protein, 9 aa, Artificial Sequence
  Synthetic Construct
QQGQTYPYT

SEQ ID NO: 49 - protein, 10 aa, Artificial Sequence
  Synthetic Construct
ESVEYYVTSL

SEQ ID NO: 50 - protein, 3 aa, Artificial Sequence
  Synthetic Construct
AAS

SEQ ID NO: 51 - protein, 9 aa, Artificial Sequence
  Synthetic Construct
QQSRKVPYT

SEQ ID NO: 52 - protein, 11 aa, Artificial Sequence
  Synthetic Construct
QSLVHNNANTY

SEQ ID NO: 53 - protein, 3 aa, Artificial Sequence
  Synthetic Construct
KVS

SEQ ID NO: 54 - protein, 7 aa, Artificial Sequence
  Synthetic Construct
GQGTQYP

SEQ ID NO: 55 - protein, 10 aa, Artificial Sequence
  Synthetic Construct
QSVDYDGDSY

SEQ ID NO: 56 - protein, 3 aa, Artificial Sequence
  Synthetic Construct
DAS

SEQ ID NO: 57 - protein, 9 aa, Artificial Sequence
  Synthetic Construct
QQSTEDPWT

SEQ ID NO: 58 - protein, 6 aa, Artificial Sequence
  Synthetic Construct
QDVSTV

SEQ ID NO: 59 - protein, 9 aa, Artificial Sequence
  Synthetic Construct
QQHYSPPYT

SEQ ID NO: 60 - protein, 450 aa, Artificial Sequence
  Synthetic Construct
EVQLVESGGGLVQPGRSLRLSCAASGFTFDDYAMHWVRQAPGKGLEWVSAITWNSGHIDYADSVEGRFTISRDNAKNSLYLQMNSLRAEDTAVYYCAKVSYLSTASSLDYWGQGTLVTVSSASTKGPSVFPLAPSSKSTSGGTAALGCLVKDYFPEPVTVSWNSGALTSGVHTFPAVLQSSGLYSLSSVVTVPSSSLGTQTYICNVNHKPSNTKVDKKVEPKSCDKTHTCPPCPAPELLGGPSVFLFPPKPKDTLMISRTPEVTCVVVDVSHEDPEVKFNWYVDGVEVHNAKTKPREEQYNSTYRVVSVLTVLHQDWLNGKEYKCKVSNKALPAPIEKTISKAKGQPREPQVCTLPPSRDELTKNQVSLSCAVKGFYPSDIAVEWESNGQPENNYKTTPPVLDSDGSFFLVSKLTVDKSRWQQGNVFSCSVMHEALHNHYTQKSLSLSPG

SEQ ID NO: 61 - protein, 213 aa, Artificial Sequence
  Synthetic Construct
DIQMTQSPSSLSASVGDRVTITCRASQGIRNYLAWYQQKPGKAPKLLIYAASTLQSGVPSRFSGSGSGTDFTLTISSLQPEDVATYYCQRYNRAPYTFGQGTKVEIKGQPKAAPSVTLFPPSSEELQANKATLVCLISDFYPGAVTVAWKADSSPVKAGVETTTPSKQSNNKYAASSYLSLTPEQWKSHRSYSCQVTHEGSTVEKTVAPTECS

SEQ ID NO: 62 - protein, 570 aa, Artificial Sequence
  Synthetic Construct
QVQLQQSGPELVKPGASVKISCKASGYSFTSYWIHWIKQRPGQGLEWIGMIDPSDGETRLNQRFQGRATLTVDESTSTAYMQLRSPTSEDSAVYYCTRLKEYGNYDSFYFDVWGAGTLVTVSSEVQLKESGPGLVAPGGSLSITCTVSGFSLTDSSINWVRQPPGKGLEWLGMIWGDGRIDYADALKSRLSISKDSSKSQVFLEMTSLRTDDTATYYCARDGYFPYAMDFWGQGTSVTVSSASTKGPSVFPLAPSSKSTSGGTAALGCLVKDYFPEPVTVSWNSGALTSGVHTFPAVLQSSGLYSLSSVVTVPSSSLGTQTYICNVNHKPSNTKVDKKVEPKSCDKTHTCPPCPAPELLGGPSVFLFPPKPKDTLMISRTPEVTCVVVDVSHEDPEVKFNWYVDGVEVHNAKTKPREEQYNSTYRVVSVLTVLHQDWLNGKEYKCKVSNKALPAPIEKTISKAKGQPREPQVYTLPPCRDELTKNQVSLWCLVKGFYPSDIAVEWESNGQPENNYKTTPPVLDSDGSFFLYSKLTVDKSRWQQGNVFSCSVMHEALHNRFTQKSLSLSPG

SEQ ID NO: 63 - protein, 345 aa, Artificial Sequence
  Synthetic Construct
DIVLTQSPASLAVSLGQRATISCRASESVDSYGQSYMHWYQQKAGQPPKLLIYLASNLESGVPARFSGSGSRTDFTLTIDPVQAEDAATYYCQQNAEDSRTFGGGTKLEIKGGSGSSGSGGDIQMTQSPASLSVSVGDTITLTCHASQNIDVWLSWFQQKPGNIPKLLIYKASNLHTGVPSRFSGSGSGTGFTLTISSLQPEDIATYYCQQAHSYPFTFGGGTKLEIKGGSGSSGSGGRTVAAPSVFIFPPSDEQLKSGTASVVCLLNNFYPREAKVQWKVDNALQSGNSQESVTEQDSKDSTYSLSSTLTLSKADYEKHKVYACEVTHQGLSSPVTKSFNRGEC

SEQ ID NO: 64 - DNA, 1350 bp, Artificial Sequence
  Synthetic Construct
gaggtgcagctggtggaaagcggcggaggactggtgcagcccggcagaagcctgagactgagctgcgccgccagcggcttcaccttcgacgactacgccatgcactgggtccgccaggcccctggcaagggcctggaatgggtgtccgccatcacctggaacagcggccacatcgactacgccgacagcgtggaaggccggttcaccatcagccgggacaacgccaagaacagcctgtacctgcagatgaacagcctgcgggccgaggacaccgccgtgtactactgcgccaaggtgtcctacctgagcaccgccagcagcctggactactggggccagggcaccctggtgacagtgtccagcgcttccaccaagggccccagcgtgttccccctggcccctagcagcaagagcacatctggcggcacagccgccctgggctgcctggtcaaggactacttccccgagcccgtgacagtgtcctggaactctggcgccctgaccagcggagtgcataccttccctgccgtgctgcagtccagcggcctgtacagcctgagcagcgtggtcacagtgcccagcagcagcctgggcacccagacctacatctgcaacgtgaaccacaagcccagcaacaccaaggtggacaagaaggtggaacccaagagctgcgacaagacccacacctgtcccccctgccctgcccctgaactgctgggcggaccctccgtgttcctgttccccccaaagcccaaggacaccctgatgatcagccggacccccgaagtgacctgcgtggtggtggacgtgtcccacgaggaccctgaagtgaagttcaattggtacgtggacggcgtggaagtgcataacgccaagaccaagcccagagaggaacagtacaacagcacctaccgggtggtgtccgtgctgaccgtgctgcaccaggactggctgaacggcaaagagtacaagtgcaaggtgtccaacaaggccctgcctgcccccatcgagaaaaccatcagcaaggccaagggccagcctagagagccccaagtctgcaccctgccccccagcagagatgagctgaccaagaaccaggtgtccctgagctgcgccgtgaagggcttctaccccagcgatatcgccgtggaatgggagagcaacggccagcccgagaacaactacaagaccaccccccctgtgctggacagcgacggctcattcttcctggtgtccaagctgacagtggacaagagccggtggcagcagggcaacgtgttcagctgcagcgtgatgcacgaggccctgcacaaccattacacccagaagtccctgagcctgagccccggc

SEQ ID NO: 65 - DNA, 639 bp, Artificial Sequence
  Synthetic Construct
gacatccagatgacccagagccccagcagcctgagcgccagcgtgggcgacagagtgaccatcacctgtcgggccagccagggcatccggaactacctggcctggtatcagcagaagcccggcaaggcccccaagctgctgatctacgccgccagcacactgcagagcggcgtgcccagcagattcagcggcagcggctccggcaccgacttcaccctgaccatcagcagcctgcagcccgaggacgtggccacctactactgccagcggtacaacagagccccctacaccttcggccagggcaccaaggtggaaatcaagggacagcccaaggctgccccctcggtcaccctgttccccccaagcagcgaggaactgcaggccaacaaggccaccctcgtgtgcctgatcagcgacttctaccctggcgccgtgaccgtggcctggaaggccgatagctctcccgtgaaggccggcgtggaaaccaccacccccagcaagcagagcaacaacaaatacgccgcctccagctacctgagcctgacccccgagcagtggaagtcccaccggtcctacagctgccaggtcacacacgagggcagcaccgtggaaaagaccgtggcccccaccgagtgcagc

SEQ ID NO: 66 - DNA, 1710 bp, Artificial Sequence
  Synthetic Construct
caggtgcagctgcagcagagcggccctgagctggtcaagcctggcgccagcgtgaagatcagctgcaaggccagcggctacagcttcaccagctactggatccactggatcaagcagcggcctggccagggcctggaatggatcggcatgatcgaccccagcgacggcgagacacggctgaaccagagattccagggcagagccaccctgaccgtggacgagagcaccagcaccgcctacatgcagctgcggagccccaccagcgaggacagcgccgtgtactactgcacccggctgaaagagtacggcaactacgacagcttctacttcgacgtgtggggagccggcaccctggtcaccgtgtccagcgaagtgcagctgaaagaaagcggccctggcctggtggcccctggcggcagcctgagcatcacctgtaccgtgtccggcttcagcctgaccgacagcagcatcaactgggtccgacagccccctggcaagggcctcgagtggctgggaatgatctggggcgacggccggatcgactacgccgacgccctgaagtcccggctgagcatcagcaaggacagcagcaagagccaggtgttcctggaaatgaccagcctgcggaccgacgacaccgccacctactactgcgccagggacggctacttcccctacgccatggatttctggggccagggcaccagcgtgaccgtgtcctctgcttccaccaagggccccagcgtgttccctctggcccctagcagcaagagcacatctggcggaacagccgccctgggctgcctggtcaaggactactttcccgagcccgtgaccgtgtcctggaactctggtgccctgacaagcggagtgcataccttccctgccgtgctgcagagcagcggcctgtactctctgagcagcgtggtcaccgtgccaagcagcagcctgggcacccagacctacatctgcaacgtgaaccacaagccctccaacaccaaggtggacaagaaggtggaacccaagagctgcgacaagacccacacctgtcctccctgtcctgcccctgaactgctgggcggaccctccgtgttcctgttccctccaaagcccaaggataccctgatgatcagccggacccctgaagtgacctgcgtggtggtggacgtgtcccacgaggatcccgaagtgaagttcaattggtacgtggacggcgtggaagtgcataacgccaagaccaagcccagagaggaacagtacaacagcacctaccgggtggtgtccgtgctgacagtgctgcaccaggactggctgaacggcaaagagtacaagtgcaaggtgtccaacaaggccctgccagcccctatcgagaaaaccatcagcaaggccaagggccagccccgcgagcctcaggtgtacacactgcctccatgccgggacgagctgaccaagaaccaggtgtccctgtggtgcctcgtgaagggcttctacccctccgatatcgccgtggaatgggagagcaacggccagcccgagaacaactacaagaccacccctcccgtgctggacagcgacggctcattcttcctgtacagcaagctgaccgtggacaagtcccggtggcagcagggcaacgtgttcagctgctctgtgatgcacgaggccctgcacaaccggttcacccagaagtccctgagcctgagccctggc

SEQ ID NO: 67 - DNA, 1035 bp, Artificial Sequence
  Synthetic Construct
gacatcgtgctgacccagagccctgccagcctggccgtgtctctgggccagagagccaccatcagctgccgggccagcgagagcgtggacagctacggccagagctacatgcactggtatcagcagaaggccggccagccccccaagctgctgatctacctggccagcaacctggaaagcggcgtgcccgccagattcagcggcagcggcagcagaaccgacttcaccctgaccatcgaccccgtgcaggccgaggacgccgccacctactactgccagcagaacgccgaggacagccggaccttcggcggaggcaccaagctggaaatcaagggcggctccggcagcagcggctctggcggcgatatccagatgacccagtcccccgcctccctgagcgtgtccgtgggcgacaccatcaccctgacatgccacgccagccagaacatcgacgtgtggctgagctggttccagcagaagcctggcaacatccctaagctgctcatctataaggcctccaacctgcacaccggcgtgcccagcaggttttccggctctggcagcggcaccggctttaccctgacaatcagcagcctgcagcccgaggatatcgccacatattactgtcagcaggcccacagctaccccttcacctttggcggcggaacaaagctcgagattaagggcggcagcggaagctccggctccggcggacgtacggtggccgctccttccgtgttcatcttccctccctccgacgagcagctgaagtccggcaccgcctccgtggtgtgtctgctgaacaacttctaccctcgggaggccaaggtgcagtggaaggtggacaacgccctgcagtccggcaactcccaggagtccgtcaccgagcaggactccaaggacagcacctactccctgtcctccaccctgaccctgtccaaggccgactacgagaagcacaaggtgtacgcctgtgaggtgacccaccagggcctgtccagccctgtgaccaagtccttcaaccggggcgagtgc

SEQ ID NO: 68 - protein, 570 aa, Artificial Sequence
  Synthetic Construct
EVQLKESGPGLVAPGGSLSITCTVSGFSLTDSSINWVRQPPGKGLEWLGMIWGDGRIDYADALKSRLSISKDSSKSQVFLEMTSLRTDDTATYYCARDGYFPYAMDFWGQGTSVTVSSQVQLQQSGPELVKPGASVKISCKASGYSFTSYWIHWIKQRPGQGLEWIGMIDPSDGETRLNQRFQGRATLTVDESTSTAYMQLRSPTSEDSAVYYCTRLKEYGNYDSFYFDVWGAGTLVTVSSASTKGPSVFPLAPSSKSTSGGTAALGCLVKDYFPEPVTVSWNSGALTSGVHTFPAVLQSSGLYSLSSVVTVPSSSLGTQTYICNVNHKPSNTKVDKKVEPKSCDKTHTCPPCPAPELLGGPSVFLFPPKPKDTLMISRTPEVTCVVVDVSHEDPEVKFNWYVDGVEVHNAKTKPREEQYNSTYRVVSVLTVLHQDWLNGKEYKCKVSNKALPAPIEKTISKAKGQPREPQVYTLPPCRDELTKNQVSLWCLVKGFYPSDIAVEWESNGQPENNYKTTPPVLDSDGSFFLYSKLTVDKSRWQQGNVFSCSVMHEALHNRFTQKSLSLSPG

SEQ ID NO: 69 - protein, 345 aa, Artificial Sequence
  Synthetic Construct
DIQMTQSPASLSVSVGDTITLTCHASQNIDVWLSWFQQKPGNIPKLLIYKASNLHTGVPSRFSGSGSGTGFTLTISSLQPEDIATYYCQQAHSYPFTFGGGTKLEIKGGSGSSGSGGDIVLTQSPASLAVSLGQRATISCRASESVDSYGQSYMHWYQQKAGQPPKLLIYLASNLESGVPARFSGSGSRTDFTLTIDPVQAEDAATYYCQQNAEDSRTFGGGTKLEIKGGSGSSGSGGRTVAAPSVFIFPPSDEQLKSGTASVVCLLNNFYPREAKVQWKVDNALQSGNSQESVTEQDSKDSTYSLSSTLTLSKADYEKHKVYACEVTHQGLSSPVTKSFNRGEC

SEQ ID NO: 70 - DNA, 1035 bp, Artificial Sequence
  Synthetic Construct
gacatccagatgacccagagccccgccagcctgagcgtgtccgtgggcgataccatcaccctgacctgccacgccagccagaacatcgacgtgtggctgagctggttccagcagaagcccggcaacatccccaagctgctgatctacaaggccagcaacctgcacaccggcgtgcccagcagattcagcggctctggcagcggcaccggctttaccctgaccatcagcagcctgcagcccgaggatatcgccacctactactgccagcaggcccacagctaccccttcaccttcggcggaggcaccaagctggaaatcaagggcggcagcggcagctccggctctggcggcgatatcgtgctgacccagtctcccgcctccctggccgtgtctctgggccagagagccaccatcagctgccgggccagcgagagcgtggacagctacggccagagctacatgcactggtatcagcagaaggccggacagccccctaaactgctcatctacctggcctccaacctggaaagcggcgtgcccgccaggttttccggcagcggctccagaaccgacttcaccctgacaatcgaccccgtgcaggccgaggacgccgccacatattactgtcagcagaacgccgaggacagcagaacctttggcggcggaacaaagctcgagattaagggcggctccggctccagcggatctggcggacgtacggtggccgctccttccgtgttcatcttccctccctccgacgagcagctgaagtccggcaccgcctccgtggtgtgtctgctgaacaacttctaccctcgggaggccaaggtgcagtggaaggtggacaacgccctgcagtccggcaactcccaggagtccgtcaccgagcaggactccaaggacagcacctactccctgtcctccaccctgaccctgtccaaggccgactacgagaagcacaaggtgtacgcctgtgaggtgacccaccagggcctgtccagccctgtgaccaagtccttcaaccggggcgagtgc

SEQ ID NO: 71 - protein, 214 aa, Artificial Sequence
  Synthetic Construct
DIQMTQSPSSLSASVGDRVTITCRASQGIRNYLAWYQQKPGKAPKLLIYAASTLQSGVPSRFSGSGSGTDFTLTISSLQPEDVATYYCQRYNRAPYTFGQGTKVEIKRTVAAPSVFIFPPSDEQLKSGTASVVCLLNNFYPREAKVQWKVDNALQSGNSQESVTEQDSKDSTYSLSSTLTLSKADYEKHKVYACEVTHQGLSSPVTKSFNRGEC

SEQ ID NO: 72 - DNA, 642 bp, Artificial Sequence
  Synthetic Construct
gacatccagatgacccagagccccagcagcctgagcgccagcgtgggcgacagagtgaccatcacctgtcgggccagccagggcatccggaactacctggcctggtatcagcagaagcccggcaaggcccccaagctgctgatctacgccgccagcacactgcagagcggcgtgcccagcagattcagcggcagcggctccggcaccgacttcaccctgaccatcagcagcctgcagcccgaggacgtggccacctactactgccagcggtacaacagagccccctacaccttcggccagggcaccaaggtggaaatcaagcgtacggtggccgctccttccgtgttcatcttccctccctccgacgagcagctgaagtccggcaccgcctccgtggtgtgtctgctgaacaacttctaccctcgggaggccaaggtgcagtggaaggtggacaacgccctgcagtccggcaactcccaggagtccgtcaccgagcaggactccaaggacagcacctactccctgtcctccaccctgaccctgtccaaggccgactacgagaagcacaaggtgtacgcctgtgaggtgacccaccagggcctgtccagccctgtgaccaagtccttcaaccggggcgagtgc

SEQ ID NO: 73 - protein, 447 aa, Artificial Sequence
  Synthetic Construct
EVQLKESGPGLVAPGGSLSITCTVSGFSLTDSSINWVRQPPGKGLEWLGMIWGDGRIDYADALKSRLSISKDSSKSQVFLEMTSLRTDDTATYYCARDGYFPYAMDFWGQGTSVTVSSASTKGPSVFPLAPSSKSTSGGTAALGCLVKDYFPEPVTVSWNSGALTSGVHTFPAVLQSSGLYSLSSVVTVPSSSLGTQTYICNVNHKPSNTKVDKKVEPKSCDKTHTCPPCPAPELLGGPSVFLFPPKPKDTLMISRTPEVTCVVVDVSHEDPEVKFNWYVDGVEVHNAKTKPREEQYNSTYRVVSVLTVLHQDWLNGKEYKCKVSNKALPAPIEKTISKAKGQPREPQVCTLPPSRDELTKNQVSLSCAVKGFYPSDIAVEWESNGQPENNYKTTPPVLDSDGSFFLVSKLTVDKSRWQQGNVFSCSVMHEALHNHYTQKSLSLSPG

SEQ ID NO: 74 - protein, 217 aa, Artificial Sequence
  Synthetic Construct
DIVLTQSPASLAVSLGQRATISCRASESVDSYGQSYMHWYQQKAGQPPKLLIYLASNLESGVPARFSGSGSRTDFTLTIDPVQAEDAATYYCQQNAEDSRTFGGGTKLEIKGQPKAAPSVTLFPPSSEELQANKATLVCLISDFYPGAVTVAWKADSSPVKAGVETTTPSKQSNNKYAASSYLSLTPEQWKSHRSYSCQVTHEGSTVEKTVAPTECS

SEQ ID NO: 75 - protein, 573 aa, Artificial Sequence
  Synthetic Construct
QVQLQQSGPELVKPGASVKISCKASGYSFTSYWIHWIKQRPGQGLEWIGMIDPSDGETRLNQRFQGRATLTVDESTSTAYMQLRSPTSEDSAVYYCTRLKEYGNYDSFYFDVWGAGTLVTVSSEVQLVESGGGLVQPGRSLRLSCAASGFTFDDYAMHWVRQAPGKGLEWVSAITWNSGHIDYADSVEGRFTISRDNAKNSLYLQMNSLRAEDTAVYYCAKVSYLSTASSLDYWGQGTLVTVSSASTKGPSVFPLAPSSKSTSGGTAALGCLVKDYFPEPVTVSWNSGALTSGVHTFPAVLQSSGLYSLSSVVTVPSSSLGTQTYICNVNHKPSNTKVDKKVEPKSCDKTHTCPPCPAPELLGGPSVFLFPPKPKDTLMISRTPEVTCVVVDVSHEDPEVKFNWYVDGVEVHNAKTKPREEQYNSTYRVVSVLTVLHQDWLNGKEYKCKVSNKALPAPIEKTISKAKGQPREPQVYTLPPCRDELTKNQVSLWCLVKGFYPSDIAVEWESNGQPENNYKTTPPVLDSDGSFFLYSKLTVDKSRWQQGNVFSCSVMHEALHNRFTQKSLSLSPG

SEQ ID NO: 76 - protein, 341 aa, Artificial Sequence
  Synthetic Construct
DIQMTQSPSSLSASVGDRVTITCRASQGIRNYLAWYQQKPGKAPKLLIYAASTLQSGVPSRFSGSGSGTDFTLTISSLQPEDVATYYCQRYNRAPYTFGQGTKVEIKGGSGSSGSGGDIQMTQSPASLSVSVGDTITLTCHASQNIDVWLSWFQQKPGNIPKLLIYKASNLHTGVPSRFSGSGSGTGFTLTISSLQPEDIATYYCQQAHSYPFTFGGGTKLEIKGGSGSSGSGGRTVAAPSVFIFPPSDEQLKSGTASVVCLLNNFYPREAKVQWKVDNALQSGNSQESVTEQDSKDSTYSLSSTLTLSKADYEKHKVYACEVTHQGLSSPVTKSFNRGEC

SEQ ID NO: 77 - DNA, 1341 bp, Artificial Sequence
  Synthetic Construct
gaggtgcagctgaaggagagcggccccggcctggtggcccccggcggcagcctgagcatcacctgcaccgtgagcggcttcagcctgaccgacagcagcatcaactgggtgcgccagccccccggcaagggcctggagtggctgggcatgatctggggcgacggccgcatcgactacgccgacgccctgaagagccgcctgagcatcagcaaggacagcagcaagagccaggtgttcctggagatgaccagcctgcgcaccgacgacaccgccacctactactgcgcccgcgacggctacttcccctacgccatggacttctggggccagggcaccagcgtgaccgtgagcagcgccagcaccaagggccccagcgtgttccccctggcccctagcagcaagagcacatctggcggcacagccgccctgggctgcctggtcaaggactacttccccgagcccgtgacagtgtcctggaactctggcgccctgaccagcggagtgcataccttccctgccgtgctgcagtccagcggcctgtacagcctgagcagcgtggtcacagtgcccagcagcagcctgggcacccagacctacatctgcaacgtgaaccacaagcccagcaacaccaaggtggacaagaaggtggaacccaagagctgcgacaagacccacacctgtcccccctgccctgcccctgaactgctgggcggaccctccgtgttcctgttccccccaaagcccaaggacaccctgatgatcagccggacccccgaagtgacctgcgtggtggtggacgtgtcccacgaggaccctgaagtgaagttcaattggtacgtggacggcgtggaagtgcataacgccaagaccaagcccagagaggaacagtacaacagcacctaccgggtggtgtccgtgctgaccgtgctgcaccaggactggctgaacggcaaagagtacaagtgcaaggtgtccaacaaggccctgcctgcccccatcgagaaaaccatcagcaaggccaagggccagcctagagagccccaagtctgcaccctgccccccagcagagatgagctgaccaagaaccaggtgtccctgagctgcgccgtgaagggcttctaccccagcgatatcgccgtggaatgggagagcaacggccagcccgagaacaactacaagaccaccccccctgtgctggacagcgacggctcattcttcctggtgtccaagctgacagtggacaagagccggtggcagcagggcaacgtgttcagctgcagcgtgatgcacgaggccctgcacaaccattacacccagaagtccctgagcctgagccccggc

SEQ ID NO: 78 - DNA, 651 bp, Artificial Sequence
  Synthetic Construct
gacatcgtgctgacccagagccctgccagcctggccgtgtctctgggccagagagccaccatcagctgccgggccagcgagagcgtggacagctacggccagagctacatgcactggtatcagcagaaggccggccagccccccaagctgctgatctacctggccagcaacctggaaagcggcgtgcccgccagattcagcggcagcggcagcagaaccgacttcaccctgaccatcgaccccgtgcaggccgaggacgccgccacctactactgccagcagaacgccgaggacagccggaccttcggcggaggcaccaagctggaaatcaagggacagcccaaggctgccccctcggtcaccctgttccccccaagcagcgaggaactgcaggccaacaaggccaccctcgtgtgcctgatcagcgacttctaccctggcgccgtgaccgtggcctggaaggccgatagctctcccgtgaaggccggcgtggaaaccaccacccccagcaagcagagcaacaacaaatacgccgccagcagctacctgagcctgacccccgagcagtggaagtcccaccggtcctacagctgccaggtcacacacgagggcagcaccgtggaaaagaccgtggcccccaccgagtgcagc

SEQ ID NO: 79 - DNA, 1719 bp, Artificial Sequence
  Synthetic Construct
caggtgcagctgcagcagagcggccctgagctggtcaagcctggcgccagcgtgaagatcagctgcaaggccagcggctacagcttcaccagctactggatccactggatcaagcagcggcctggccagggcctggaatggatcggcatgatcgaccccagcgacggcgagacacggctgaaccagagattccagggcagagccaccctgaccgtggacgagagcaccagcaccgcctacatgcagctgcggagccccaccagcgaggacagcgccgtgtactactgcacccggctgaaagagtacggcaactacgacagcttctacttcgacgtgtggggagccggcaccctggtcaccgtgtccagcgaagtgcagctggtggaaagcggcggaggcctggtgcagcccggcagaagcctgagactgagctgcgccgccagcggcttcaccttcgacgactacgccatgcactgggtccgacaggcccctggcaaaggactggaatgggtgtccgccatcacctggaacagcggccacatcgactacgccgacagcgtggaaggccggttcaccatcagccgggacaacgccaagaacagcctgtacctgcagatgaacagcctgcgggccgaggataccgccgtgtattattgcgccaaggtgtcctacctgagcaccgccagcagcctggactactggggccagggcaccctcgtgacagtgtcctccgcttccaccaagggccccagcgtgttccctctggcccctagcagcaagagcacatctggcggaacagccgccctgggctgcctggtcaaggactactttcccgagcccgtgaccgtgtcctggaactctggtgccctgacaagcggagtgcataccttccctgccgtgctgcagagcagcggcctgtactctctgagcagcgtggtcaccgtgccaagcagcagcctgggcacccagacctacatctgcaacgtgaaccacaagccctccaacaccaaggtggacaagaaggtggaacccaagagctgcgacaagacccacacctgtcctccctgtcctgcccctgaactgctgggcggaccctccgtgttcctgttccctccaaagcccaaggataccctgatgatcagccggacccctgaagtgacctgcgtggtggtggacgtgtcccacgaggatcccgaagtgaagttcaattggtacgtggacggcgtggaagtgcataacgccaagaccaagcccagagaggaacagtacaacagcacctaccgggtggtgtccgtgctgacagtgctgcaccaggactggctgaacggcaaagagtacaagtgcaaggtgtccaacaaggccctgccagcccctatcgagaaaaccatcagcaaggccaagggccagccccgcgagcctcaggtgtacacactgcctccatgccgggacgagctgaccaagaaccaggtgtccctgtggtgcctcgtgaagggcttctacccctccgatatcgccgtggaatgggagagcaacggccagcccgagaacaactacaagaccacccctcccgtgctggacagcgacggctcattcttcctgtacagcaagctgaccgtggacaagtcccggtggcagcagggcaacgtgttcagctgctctgtgatgcacgaggccctgcacaaccggttcacccagaagtccctgagcctgagccctggc

SEQ ID NO: 80 - DNA, 1023 bp, Artificial Sequence
  Synthetic Construct
gacatccagatgacccagagccccagcagcctgagcgccagcgtgggcgacagagtgaccatcacctgtcgggccagccagggcatccggaactacctggcctggtatcagcagaagcccggcaaggcccccaagctgctgatctacgccgccagcacactgcagagcggcgtgcccagcagattcagcggcagcggctccggcaccgacttcaccctgaccatcagcagcctgcagcccgaggacgtggccacctactactgccagcggtacaacagagccccctacaccttcggccagggcaccaaggtggaaatcaagggcggctctggcagctccggcagcggcggagacattcagatgacacagtcccccgccagcctgtccgtgtccgtgggcgataccatcaccctgacatgccacgccagccagaacatcgacgtgtggctgagctggttccagcagaaacctggcaacatccctaagctgctcatctataaggccagcaacctgcacacaggcgtgccctccagattctccggctctggctctggcaccggctttacactgacaatcagttctctgcagcctgaggatatcgccacatattactgtcagcaggcccacagctaccctttcaccttcggaggcggcaccaagctcgagattaagggcggaagcggctcctccggctccggcggacgtacggtggccgctccttccgtgttcatcttccctccctccgacgagcagctgaagtccggcaccgcctccgtggtgtgtctgctgaacaacttctaccctcgggaggccaaggtgcagtggaaggtggacaacgccctgcagtccggcaactcccaggagtccgtcaccgagcaggactccaaggacagcacctactccctgtcctccaccctgaccctgtccaaggccgactacgagaagcacaaggtgtacgcctgtgaggtgacccaccagggcctgtccagccctgtgaccaagtccttcaaccggggcgagtgc

SEQ ID NO: 81 - protein, 573 aa, Artificial Sequence
  Synthetic Construct
EVQLVESGGGLVQPGRSLRLSCAASGFTFDDYAMHWVRQAPGKGLEWVSAITWNSGHIDYADSVEGRFTISRDNAKNSLYLQMNSLRAEDTAVYYCAKVSYLSTASSLDYWGQGTLVTVSSQVQLQQSGPELVKPGASVKISCKASGYSFTSYWIHWIKQRPGQGLEWIGMIDPSDGETRLNQRFQGRATLTVDESTSTAYMQLRSPTSEDSAVYYCTRLKEYGNYDSFYFDVWGAGTLVTVSSASTKGPSVFPLAPSSKSTSGGTAALGCLVKDYFPEPVTVSWNSGALTSGVHTFPAVLQSSGLYSLSSVVTVPSSSLGTQTYICNVNHKPSNTKVDKKVEPKSCDKTHTCPPCPAPELLGGPSVFLFPPKPKDTLMISRTPEVTCVVVDVSHEDPEVKFNWYVDGVEVHNAKTKPREEQYNSTYRVVSVLTVLHQDWLNGKEYKCKVSNKALPAPIEKTISKAKGQPREPQVYTLPPCRDELTKNQVSLWCLVKGFYPSDIAVEWESNGQPENNYKTTPPVLDSDGSFFLYSKLTVDKSRWQQGNVFSCSVMHEALHNRFTQKSLSLSPG

SEQ ID NO: 82 - protein, 341 aa, Artificial Sequence
  Synthetic Construct
DIQMTQSPASLSVSVGDTITLTCHASQNIDVWLSWFQQKPGNIPKLLIYKASNLHTGVPSRFSGSGSGTGFTLTISSLQPEDIATYYCQQAHSYPFTFGGGTKLEIKGGSGSSGSGGDIQMTQSPSSLSASVGDRVTITCRASQGIRNYLAWYQQKPGKAPKLLIYAASTLQSGVPSRFSGSGSGTDFTLTISSLQPEDVATYYCQRYNRAPYTFGQGTKVEIKGGSGSSGSGGRTVAAPSVFIFPPSDEQLKSGTASVVCLLNNFYPREAKVQWKVDNALQSGNSQESVTEQDSKDSTYSLSSTLTLSKADYEKHKVYACEVTHQGLSSPVTKSFNRGEC

SEQ ID NO: 83 - DNA, 1719 bp, Artificial Sequence
  Synthetic Construct
gaggtgcagctggtggaaagcggcggaggactggtgcagcccggcagaagcctgagactgagctgcgccgccagcggcttcaccttcgacgactacgccatgcactgggtccgacaggcccctggcaagggcctggaatgggtgtccgccatcacctggaacagcggccacatcgactacgccgacagcgtggaaggccggttcaccatcagccgggacaacgccaagaacagcctgtacctgcagatgaacagcctgcgggccgaggacaccgccgtgtactactgcgccaaggtgtcctacctgagcaccgccagcagcctggactactggggccagggcaccctggtcaccgtgtccagtcaggtccagctgcagcagagcggccctgagctggtcaagcctggcgccagcgtgaagatcagctgcaaggccagcggctacagcttcaccagctactggatccactggatcaagcagcggcctggccagggcctcgagtggatcggcatgatcgaccccagcgacggcgagacacggctgaaccagagattccagggcagagccaccctgaccgtggacgagagcaccagcaccgcctacatgcagctgcggagccccaccagcgaggatagcgccgtgtattattgcacccggctgaaagagtacggcaactacgacagcttctacttcgacgtgtggggagccggcaccctcgtgacagtgtcctccgcttccaccaagggccccagcgtgttccctctggcccctagcagcaagagcacatctggcggaacagccgccctgggctgcctggtcaaggactactttcccgagcccgtgaccgtgtcctggaactctggtgccctgacaagcggagtgcataccttccctgccgtgctgcagagcagcggcctgtactctctgagcagcgtggtcaccgtgccaagcagcagcctgggcacccagacctacatctgcaacgtgaaccacaagccctccaacaccaaggtggacaagaaggtggaacccaagagctgcgacaagacccacacctgtcctccctgtcctgcccctgaactgctgggcggaccctccgtgttcctgttccctccaaagcccaaggataccctgatgatcagccggacccctgaagtgacctgcgtggtggtggacgtgtcccacgaggatcccgaagtgaagttcaattggtacgtggacggcgtggaagtgcataacgccaagaccaagcccagagaggaacagtacaacagcacctaccgggtggtgtccgtgctgacagtgctgcaccaggactggctgaacggcaaagagtacaagtgcaaggtgtccaacaaggccctgccagcccctatcgagaaaaccatcagcaaggccaagggccagccccgcgagcctcaggtgtacacactgcctccatgccgggacgagctgaccaagaaccaggtgtccctgtggtgcctcgtgaagggcttctacccctccgatatcgccgtggaatgggagagcaacggccagcccgagaacaactacaagaccacccctcccgtgctggacagcgacggctcattcttcctgtacagcaagctgaccgtggacaagtcccggtggcagcagggcaacgtgttcagctgctctgtgatgcacgaggccctgcacaaccggttcacccagaagtccctgagcctgagccctggc

SEQ ID NO: 84 - DNA, 1023 bp, Artificial Sequence
  Synthetic Construct
gacatccagatgacccagagccccgccagcctgagcgtgtccgtgggcgataccatcaccctgacctgccacgccagccagaacatcgacgtgtggctgagctggttccagcagaagcccggcaacatccccaagctgctgatctacaaggccagcaacctgcacaccggcgtgcccagcagattcagcggctctggcagcggcaccggctttaccctgaccatcagcagcctgcagcccgaggatatcgccacctactactgccagcaggcccacagctaccccttcaccttcggcggaggcaccaagctggaaatcaagggcggcagcggcagctccggcagcggcggagacattcagatgacacagtcccccagcagcctgtccgccagcgtgggcgacagagtgaccatcacctgtcgggccagccagggcatccggaactacctggcctggtatcagcagaaacctggcaaggcccctaaactgctcatctacgccgccagcacactgcagtctggcgtgccctccagattctccggaagcggctccggcaccgatttcaccctgacaatctcatctctgcagcctgaggacgtggccacatattactgccagagatacaacagagccccctacacctttggccagggcaccaaggtcgagattaagggcggatccggctccagcggcagcggaggacgtacggtggccgctccttccgtgttcatcttccctccctccgacgagcagctgaagtccggcaccgcctccgtggtgtgtctgctgaacaacttctaccctcgggaggccaaggtgcagtggaaggtggacaacgccctgcagtccggcaactcccaggagtccgtcaccgagcaggactccaaggacagcacctactccctgtcctccaccctgaccctgtccaaggccgactacgagaagcacaaggtgtacgcctgtgaggtgacccaccagggcctgtccagccctgtgaccaagtccttcaaccggggcgagtgc

SEQ ID NO: 85 - protein, 452 aa, Artificial Sequence
  Synthetic Construct
QVQLQQSGPELVKPGASVKISCKASGYSFTSYWIHWIKQRPGQGLEWIGMIDPSDGETRLNQRFQGRATLTVDESTSTAYMQLRSPTSEDSAVYYCTRLKEYGNYDSFYFDVWGAGTLVTVSSASTKGPSVFPLAPSSKSTSGGTAALGCLVKDYFPEPVTVSWNSGALTSGVHTFPAVLQSSGLYSLSSVVTVPSSSLGTQTYICNVNHKPSNTKVDKKVEPKSCDKTHTCPPCPAPELLGGPSVFLFPPKPKDTLMISRTPEVTCVVVDVSHEDPEVKFNWYVDGVEVHNAKTKPREEQYNSTYRVVSVLTVLHQDWLNGKEYKCKVSNKALPAPIEKTISKAKGQPREPQVCTLPPSRDELTKNQVSLSCAVKGFYPSDIAVEWESNGQPENNYKTTPPVLDSDGSFFLVSKLTVDKSRWQQGNVFSCSVMHEALHNHYTQKSLSLSPG

SEQ ID NO: 86 - protein, 213 aa, Artificial Sequence
  Synthetic Construct
DIQMTQSPASLSVSVGDTITLTCHASQNIDVWLSWFQQKPGNIPKLLIYKASNLHTGVPSRFSGSGSGTGFTLTISSLQPEDIATYYCQQAHSYPFTFGGGTKLEIKGQPKAAPSVTLFPPSSEELQANKATLVCLISDFYPGAVTVAWKADSSPVKAGVETTTPSKQSNNKYAASSYLSLTPEQWKSHRSYSCQVTHEGSTVEKTVAPTECS

SEQ ID NO: 87 - protein, 568 aa, Artificial Sequence
  Synthetic Construct
EVQLKESGPGLVAPGGSLSITCTVSGFSLTDSSINWVRQPPGKGLEWLGMIWGDGRIDYADALKSRLSISKDSSKSQVFLEMTSLRTDDTATYYCARDGYFPYAMDFWGQGTSVTVSSEVQLVESGGGLVQPGRSLRLSCAASGFTFDDYAMHWVRQAPGKGLEWVSAITWNSGHIDYADSVEGRFTISRDNAKNSLYLQMNSLRAEDTAVYYCAKVSYLSTASSLDYWGQGTLVTVSSASTKGPSVFPLAPSSKSTSGGTAALGCLVKDYFPEPVTVSWNSGALTSGVHTFPAVLQSSGLYSLSSVVTVPSSSLGTQTYICNVNHKPSNTKVDKKVEPKSCDKTHTCPPCPAPELLGGPSVFLFPPKPKDTLMISRTPEVTCVVVDVSHEDPEVKFNWYVDGVEVHNAKTKPREEQYNSTYRVVSVLTVLHQDWLNGKEYKCKVSNKALPAPIEKTISKAKGQPREPQVYTLPPCRDELTKNQVSLWCLVKGFYPSDIAVEWESNGQPENNYKTTPPVLDSDGSFFLYSKLTVDKSRWQQGNVFSCSVMHEALHNRFTQKSLSLSPG

SEQ ID NO: 88 - protein, 344 aa, Artificial Sequence
  Synthetic Construct
IQMTQSPSSLSASVGDRVTITCRASQGIRNYLAWYQQKPGKAPKLLIYAASTLQSGVPSRFSGSGSGTDFTLTISSLQPEDVATYYCQRYNRAPYTFGQGTKVEIKGGSGSSGSGGDIVLTQSPASLAVSLGQRATISCRASESVDSYGQSYMHWYQQKAGQPPKLLIYLASNLESGVPARFSGSGSRTDFTLTIDPVQAEDAATYYCQQNAEDSRTFGGGTKLEIKGGSGSSGSGGRTVAAPSVFIFPPSDEQLKSGTASVVCLLNNFYPREAKVQWKVDNALQSGNSQESVTEQDSKDSTYSLSSTLTLSKADYEKHKVYACEVTHQGLSSPVTKSFNRGEC

SEQ ID NO: 89 - DNA, 1356 bp, Artificial Sequence
  Synthetic Construct
caggtgcagctgcagcagagcggccccgagctggtgaagcccggcgccagcgtgaagatcagctgcaaggccagcggctacagcttcaccagctactggattcactggatcaagcagcgccccggccagggcctggagtggatcggcatgatcgaccccagcgacggcgagacccgcctgaaccagcgcttccagggccgcgccaccctgaccgtggacgagagcaccagcaccgcctacatgcagctgcgcagccccaccagcgaggacagcgccgtgtactactgcacccgcctgaaggagtacggcaactacgacagcttctacttcgacgtgtggggcgccggcaccctggtgaccgtgagcagcgccagcaccaagggccccagcgtgttccccctggcccctagcagcaagagcacatctggcggcacagccgccctgggctgcctggtcaaggactacttccccgagcccgtgacagtgtcctggaactctggcgccctgaccagcggagtgcataccttccctgccgtgctgcagtccagcggcctgtacagcctgagcagcgtggtcacagtgcccagcagcagcctgggcacccagacctacatctgcaacgtgaaccacaagcccagcaacaccaaggtggacaagaaggtggaacccaagagctgcgacaagacccacacctgtcccccctgccctgcccctgaactgctgggcggaccctccgtgttcctgttccccccaaagcccaaggacaccctgatgatcagccggacccccgaagtgacctgcgtggtggtggacgtgtcccacgaggaccctgaagtgaagttcaattggtacgtggacggcgtggaagtgcataacgccaagaccaagcccagagaggaacagtacaacagcacctaccgggtggtgtccgtgctgaccgtgctgcaccaggactggctgaacggcaaagagtacaagtgcaaggtgtccaacaaggccctgcctgcccccatcgagaaaaccatcagcaaggccaagggccagcctagagagccccaagtctgcaccctgccccccagcagagatgagctgaccaagaaccaggtgtccctgagctgcgccgtgaagggcttctaccccagcgatatcgccgtggaatgggagagcaacggccagcccgagaacaactacaagaccaccccccctgtgctggacagcgacggctcattcttcctggtgtccaagctgacagtggacaagagccggtggcagcagggcaacgtgttcagctgcagcgtgatgcacgaggccctgcacaaccattacacccagaagtccctgagcctgagccccggc

SEQ ID NO: 90 - DNA, 639 bp, Artificial Sequence
  Synthetic Construct
gacatccagatgacccagagccccgccagcctgagcgtgtccgtgggcgataccatcaccctgacctgccacgccagccagaacatcgacgtgtggctgagctggttccagcagaagcccggcaacatccccaagctgctgatctacaaggccagcaacctgcacaccggcgtgcccagcagattcagcggctctggcagcggcaccggctttaccctgaccatcagcagcctgcagcccgaggatatcgccacctactactgccagcaggcccacagctaccccttcaccttcggcggaggcaccaagctggaaatcaagggacagcccaaggctgccccctcggtcaccctgttccccccaagctctgaggaactgcaggccaacaaggccaccctcgtgtgcctgatcagcgacttctaccctggcgccgtgaccgtggcctggaaggccgatagctctcccgtgaaggccggcgtggaaaccaccacccccagcaagcagagcaacaacaaatacgccgccagcagctacctgagcctgacccccgagcagtggaagtcccaccggtcctacagctgccaggtcacacacgagggcagcaccgtggaaaagaccgtggcccccaccgagtgcagc

SEQ ID NO: 91 - DNA, 1704 bp, Artificial Sequence
  Synthetic Construct
gaggtgcagctgaaagagtccggccctggactggtggcccctggcggcagcctgagcatcacctgtaccgtgtccggcttcagcctgaccgacagcagcatcaactgggtccgacagccccctggcaagggcctggaatggctgggcatgatctggggcgacggccggatcgactacgccgacgccctgaagtcccggctgagcatcagcaaggacagcagcaagagccaggtgttcctggaaatgaccagcctgcggaccgacgacaccgccacctactactgcgccagggacggctacttcccctacgccatggatttctggggccagggcaccagcgtgaccgtgtcctccgaagtgcagctggtggaaagcggcggaggcctggtgcagcccggcagaagcctgagactgagctgcgccgccagcggcttcaccttcgacgactacgccatgcactgggtccgccaggctcccggaaagggactcgagtgggtgtccgccatcacctggaacagcggccacatcgattacgccgatagcgtggaaggccggttcaccatcagccgggacaacgccaagaacagcctgtacctgcagatgaacagcctgagagccgaggataccgccgtgtactactgtgccaaggtgtcctacctgagcaccgccagcagcctggactactggggacagggaaccctggtcaccgtgtccagcgcttccaccaagggccccagcgtgttccctctggcccctagcagcaagagcacatctggcggaacagccgccctgggctgcctggtcaaggactactttcccgagcccgtgaccgtgtcctggaactctggtgccctgacaagcggagtgcataccttccctgccgtgctgcagagcagcggcctgtactctctgagcagcgtggtcaccgtgccaagcagcagcctgggcacccagacctacatctgcaacgtgaaccacaagccctccaacaccaaggtggacaagaaggtggaacccaagagctgcgacaagacccacacctgtcctccctgtcctgcccctgaactgctgggcggaccctccgtgttcctgttccctccaaagcccaaggataccctgatgatcagccggacccctgaagtgacctgcgtggtggtggacgtgtcccacgaggatcccgaagtgaagttcaattggtacgtggacggcgtggaagtgcataacgccaagaccaagcccagagaggaacagtacaacagcacctaccgggtggtgtccgtgctgacagtgctgcaccaggactggctgaacggcaaagagtacaagtgcaaggtgtccaacaaggccctgccagcccctatcgagaaaaccatcagcaaggccaagggccagccccgcgagcctcaggtgtacacactgcctccatgccgggacgagctgaccaagaaccaggtgtccctgtggtgcctcgtgaagggcttctacccctccgatatcgccgtggaatgggagagcaacggccagcccgagaacaactacaagaccacccctcccgtgctggacagcgacggctcattcttcctgtacagcaagctgaccgtggacaagtcccggtggcagcagggcaacgtgttcagctgctctgtgatgcacgaggccctgcacaaccggttcacccagaagtccctgagcctgagccctggc

SEQ ID NO: 92 - DNA, 1035 bp, Artificial Sequence
  Synthetic Construct
gacatccagatgacccagagccccagcagcctgagcgccagcgtgggcgacagagtgaccatcacctgtcgggccagccagggcatccggaactacctggcctggtatcagcagaagcccggcaaggcccccaagctgctgatctacgccgccagcacactgcagagcggcgtgcccagcagattcagcggcagcggctccggcaccgacttcaccctgaccatcagcagcctgcagcccgaggacgtggccacctactactgccagcggtacaacagagccccctacaccttcggccagggcaccaaggtggaaatcaagggcggctctggcagctccggctctggcggcgatatcgtgctgacccagtctcccgccagcctggccgtgtctctgggccagagagccaccatcagctgcagagccagcgagagcgtggacagctacggccagagctacatgcattggtatcagcagaaagccggccagcctcctaaactgctcatctacctggccagcaacctggaatccggcgtgcccgccaggttttccggcagcggcagcagaaccgatttcacactgacaatcgaccccgtgcaggccgaggatgccgccacatattactgtcagcagaacgccgaggacagccggaccttcggcggaggcaccaagctcgagattaagggcggaagcggctccagcggcagtggcggacgtacggtggccgctccttccgtgttcatcttccctccctccgacgagcagctgaagtccggcaccgcctccgtggtgtgtctgctgaacaacttctaccctcgggaggccaaggtgcagtggaaggtggacaacgccctgcagtccggcaactcccaggagtccgtcaccgagcaggactccaaggacagcacctactccctgtcctccaccctgaccctgtccaaggccgactacgagaagcacaaggtgtacgcctgtgaggtgacccaccagggcctgtccagccctgtgaccaagtccttcaaccggggcgagtgc

SEQ ID NO: 93 - protein, 568 aa, Artificial Sequence
  Synthetic Construct
EVQLVESGGGLVQPGRSLRLSCAASGFTFDDYAMHWVRQAPGKGLEWVSAITWNSGHIDYADSVEGRFTISRDNAKNSLYLQMNSLRAEDTAVYYCAKVSYLSTASSLDYWGQGTLVTVSSEVQLKESGPGLVAPGGSLSITCTVSGFSLTDSSINWVRQPPGKGLEWLGMIWGDGRIDYADALKSRLSISKDSSKSQVFLEMTSLRTDDTATYYCARDGYFPYAMDFWGQGTSVTVSSASTKGPSVFPLAPSSKSTSGGTAALGCLVKDYFPEPVTVSWNSGALTSGVHTFPAVLQSSGLYSLSSVVTVPSSSLGTQTYICNVNHKPSNTKVDKKVEPKSCDKTHTCPPCPAPELLGGPSVFLFPPKPKDTLMISRTPEVTCVVVDVSHEDPEVKFNWYVDGVEVHNAKTKPREEQYNSTYRVVSVLTVLHQDWLNGKEYKCKVSNKALPAPIEKTISKAKGQPREPQVYTLPPCRDELTKNQVSLWCLVKGFYPSDIAVEWESNGQPENNYKTTPPVLDSDGSFFLYSKLTVDKSRWQQGNVFSCSVMHEALHNRFTQKSLSLSPG

SEQ ID NO: 94 - protein, 345 aa, Artificial Sequence
  Synthetic Construct
DIVLTQSPASLAVSLGQRATISCRASESVDSYGQSYMHWYQQKAGQPPKLLIYLASNLESGVPARFSGSGSRTDFTLTIDPVQAEDAATYYCQQNAEDSRTFGGGTKLEIKGGSGSSGSGGDIQMTQSPSSLSASVGDRVTITCRASQGIRNYLAWYQQKPGKAPKLLIYAASTLQSGVPSRFSGSGSGTDFTLTISSLQPEDVATYYCQRYNRAPYTFGQGTKVEIKGGSGSSGSGGRTVAAPSVFIFPPSDEQLKSGTASVVCLLNNFYPREAKVQWKVDNALQSGNSQESVTEQDSKDSTYSLSSTLTLSKADYEKHKVYACEVTHQGLSSPVTKSFNRGEC

SEQ ID NO: 95 - DNA, 1704 bp, Artificial Sequence
  Synthetic Construct
gaggtgcagctggtggaaagcggcggaggactggtgcagcccggcagaagcctgagactgagctgcgccgccagcggcttcaccttcgacgactacgccatgcactgggtccgacaggcccctggcaagggcctggaatgggtgtccgccatcacctggaacagcggccacatcgactacgccgacagcgtggaaggccggttcaccatcagccgggacaacgccaagaacagcctgtacctgcagatgaacagcctgcgggccgaggacaccgccgtgtactactgcgccaaggtgtcctacctgagcaccgccagcagcctggactactggggccagggcaccctggtcaccgtgtcctccgaagtgcagctgaaagagtccggccctggcctggtggcccctggcggcagcctgagcatcacctgtaccgtgtccggcttcagcctgaccgacagcagcatcaactgggtccgccagcctcccggaaagggactcgagtggctgggcatgatctggggcgacggccggatcgattacgccgatgccctgaagtcccggctgagcatcagcaaggacagcagcaagagccaggtgttcctggaaatgaccagcctgagaaccgacgacaccgccacctactactgtgcccgggacggctacttcccctacgccatggatttctggggacagggaaccagcgtgaccgtgtccagcgcttccaccaagggccccagcgtgttccctctggcccctagcagcaagagcacatctggcggaacagccgccctgggctgcctggtcaaggactactttcccgagcccgtgaccgtgtcctggaactctggtgccctgacaagcggagtgcataccttccctgccgtgctgcagagcagcggcctgtactctctgagcagcgtggtcaccgtgccaagcagcagcctgggcacccagacctacatctgcaacgtgaaccacaagccctccaacaccaaggtggacaagaaggtggaacccaagagctgcgacaagacccacacctgtcctccctgtcctgcccctgaactgctgggcggaccctccgtgttcctgttccctccaaagcccaaggataccctgatgatcagccggacccctgaagtgacctgcgtggtggtggacgtgtcccacgaggatcccgaagtgaagttcaattggtacgtggacggcgtggaagtgcataacgccaagaccaagcccagagaggaacagtacaacagcacctaccgggtggtgtccgtgctgacagtgctgcaccaggactggctgaacggcaaagagtacaagtgcaaggtgtccaacaaggccctgccagcccctatcgagaaaaccatcagcaaggccaagggccagccccgcgagcctcaggtgtacacactgcctccatgccgggacgagctgaccaagaaccaggtgtccctgtggtgcctcgtgaagggcttctacccctccgatatcgccgtggaatgggagagcaacggccagcccgagaacaactacaagaccacccctcccgtgctggacagcgacggctcattcttcctgtacagcaagctgaccgtggacaagtcccggtggcagcagggcaacgtgttcagctgctctgtgatgcacgaggccctgcacaaccggttcacccagaagtccctgagcctgagccctggc

SEQ ID NO: 96 - DNA, 1035 bp, Artificial Sequence
  Synthetic Construct
gacatcgtgctgacccagagccctgccagcctggccgtgtctctgggccagagagccaccatcagctgccgggccagcgagagcgtggacagctacggccagagctacatgcactggtatcagcagaaggccggccagccccccaagctgctgatctacctggccagcaacctggaaagcggcgtgcccgccagattcagcggcagcggcagcagaaccgacttcaccctgaccatcgaccccgtgcaggccgaggacgccgccacctactactgccagcagaacgccgaggacagccggaccttcggcggaggcaccaagctggaaatcaagggcggctccggcagcagcggctctggcggcgatatccagatgacccagtcccccagcagcctgagcgccagcgtgggcgacagagtgaccatcacctgtagagccagccagggcatccggaactacctggcttggtatcagcagaaacccggaaaggcccctaaactgctcatctacgccgccagcaccctgcagtccggcgtgccaagcagattctccggctctggcagcggcaccgatttcacactgacaatcagcagcctgcagcccgaggatgtggccacctattattgccagagatacaacagagccccctacaccttcggccagggcaccaaggtcgagattaagggcggaagcggcagctccggctccggcggacgtacggtggccgctccttccgtgttcatcttccctccctccgacgagcagctgaagtccggcaccgcctccgtggtgtgtctgctgaacaacttctaccctcgggaggccaaggtgcagtggaaggtggacaacgccctgcagtccggcaactcccaggagtccgtcaccgagcaggactccaaggacagcacctactccctgtcctccaccctgaccctgtccaaggccgactacgagaagcacaaggtgtacgcctgtgaggtgacccaccagggcctgtccagccctgtgaccaagtccttcaaccggggcgagtgc

SEQ ID NO: 97 - DNA, 1710 bp, Artificial Sequence
  Synthetic Construct
gaggtgcagctgaaagagtccggccctggactggtggcccctggcggcagcctgagcatcacctgtaccgtgtccggcttcagcctgaccgacagcagcatcaactgggtccgacagccccctggcaagggcctggaatggctgggcatgatctggggcgacggccggatcgactacgccgacgccctgaagtcccggctgagcatcagcaaggacagcagcaagagccaggtgttcctggaaatgaccagcctgcggaccgacgacaccgccacctactactgcgccagggacggctacttcccctacgccatggatttctggggccagggcaccagcgtgaccgtgtccagtcaggtccagctgcagcagagcggccctgagctggtcaagcctggcgccagcgtgaagatcagctgcaaggccagcggctacagcttcaccagctactggatccactggatcaagcagcggcctggccagggcctcgagtggatcggaatgatcgaccccagcgacggcgagacacggctgaaccagagattccagggcagagccaccctgaccgtggacgagagcaccagcaccgcctacatgcagctgcggagccccaccagcgaggacagcgccgtgtactactgcacccggctgaaagaatacggcaactacgacagcttctacttcgacgtgtggggagccggcaccctggtcaccgtgtctagcgcttccaccaagggccccagcgtgttccctctggcccctagcagcaagagcacatctggcggaacagccgccctgggctgcctggtcaaggactactttcccgagcccgtgaccgtgtcctggaactctggtgccctgacaagcggagtgcataccttccctgccgtgctgcagagcagcggcctgtactctctgagcagcgtggtcaccgtgccaagcagcagcctgggcacccagacctacatctgcaacgtgaaccacaagccctccaacaccaaggtggacaagaaggtggaacccaagagctgcgacaagacccacacctgtcctccctgtcctgcccctgaactgctgggcggaccctccgtgttcctgttccctccaaagcccaaggataccctgatgatcagccggacccctgaagtgacctgcgtggtggtggacgtgtcccacgaggatcccgaagtgaagttcaattggtacgtggacggcgtggaagtgcataacgccaagaccaagcccagagaggaacagtacaacagcacctaccgggtggtgtccgtgctgacagtgctgcaccaggactggctgaacggcaaagagtacaagtgcaaggtgtccaacaaggccctgccagcccctatcgagaaaaccatcagcaaggccaagggccagccccgcgagcctcaggtgtacacactgcctccatgccgggacgagctgaccaagaaccaggtgtccctgtggtgcctcgtgaagggcttctacccctccgatatcgccgtggaatgggagagcaacggccagcccgagaacaactacaagaccacccctcccgtgctggacagcgacggctcattcttcctgtacagcaagctgaccgtggacaagtcccggtggcagcagggcaacgtgttcagctgctctgtgatgcacgaggccctgcacaaccggttcacccagaagtccctgagcctgagccctggc

SEQ ID NO: 98 - protein, 4 aa, Artificial Sequence
  Synthetic Construct
GGGG

SEQ ID NO: 99 - protein, 5 aa, Artificial Sequence
  Synthetic Construct
GGGGG

SEQ ID NO: 100 - protein, 6 aa, Artificial Sequence
  Synthetic Construct
GGGGGG

SEQ ID NO: 101 - protein, 7 aa, Artificial Sequence
  Synthetic Construct
GGGGGGG

SEQ ID NO: 102 - protein, 8 aa, Artificial Sequence
  Synthetic Construct
GGGGGGGG

SEQ ID NO: 103 - protein, 5 aa, Artificial Sequence
  Synthetic Construct
GGGGS

SEQ ID NO: 104 - protein, 10 aa, Artificial Sequence
  Synthetic Construct
GGGGSGGGGS

SEQ ID NO: 105 - protein, 15 aa, Artificial Sequence
  Synthetic Construct
GGGGSGGGGSGGGGS

SEQ ID NO: 106 - protein, 5 aa, Artificial Sequence
  Synthetic Construct
TKGPS

SEQ ID NO: 107 - protein, 5 aa, Artificial Sequence
  Synthetic Construct
TVAAP

SEQ ID NO: 108 - protein, 5 aa, Artificial Sequence
  Synthetic Construct
QPKAA

SEQ ID NO: 109 - protein, 5 aa, Artificial Sequence
  Synthetic Construct
QRIEG

SEQ ID NO: 110 - protein, 7 aa, Artificial Sequence
  Synthetic Construct
ASTKGPS

SEQ ID NO: 111 - protein, 7 aa, Artificial Sequence
  Synthetic Construct
RTVAAPS

SEQ ID NO: 112 - protein, 7 aa, Artificial Sequence
  Synthetic Construct
GQPKAAP

SEQ ID NO: 113 - protein, 7 aa, Artificial Sequence
  Synthetic Construct
HIDSPNK

SEQ ID NO: 114 - protein, 448 aa, Artificial Sequence
  Synthetic Construct
QVQLQQPGAELVKPGASVKMSCKASGYTFTSYNMHWVKQTPGRGLEWIGAIYPGNGDTSYNQKFKGKATLTADKSSSTAYMQLSSLTSEDSAVYYCARSTYYGGDWYFNVWGAGTTVTVSAASTKGPSVFPLAPCSRSTSESTAALGCLVKDYFPEPVTVSWNSGALTSGVHTFPAVLQSSGLYSLSSVVTVPSSSLGTKTYTCNVDHKPSNTKVDKRVESKYGPPCPPCPAPEFLGGPSVFLFPPKPKDTLMISRTPEVTCVVVDVSQEDPEVQFNWYVDGVEVHNAKTKPREEQFNSTYRVVSVLTVLHQDWLNGKEYKCKVSNKGLPSSIEKTISKAKGQPREPQVYTLPPCQEEMTKNQVSLWCLVKGFYPSDIAVEWESNGQPENNYKTTPPVLDSDGSFFLYSKLTVDKSRWQEGNVFSCSVMHEALHNHYTQKSLSLSLGK

SEQ ID NO: 115 - protein, 213 aa, Artificial Sequence
  Synthetic Construct
QIVLSQSPAILSASPGEKVTMTCRASSSVSYIHWFQQKPGSSPKPWIYATSNLASGVPVRFSGSGSGTSYSLTISRVEAEDAATYYCQQWTSNPPTFGGGTKLEIKRTVAAPSVFIFPPSDEQLKSGTASVVCLLNNFYPREAKVQWKVDNALQSGNSQESVTEQDSKDSTYSLSSTLTLSKADYEKHKVYACEVTHQGLSSPVTKSFNRGEC

SEQ ID NO: 116 - DNA, 1344 bp, Artificial Sequence
  Synthetic Construct
caggtgcagctgcagcagcctggcgccgaactcgtgaaacctggcgcctccgtgaagatgagctgcaaggccagcggctacaccttcaccagctacaacatgcactgggtcaagcagacccccggcagaggcctggaatggatcggcgccatctaccccggcaacggcgacacctcctacaaccagaagttcaagggcaaggccaccctgaccgccgacaagagcagcagcacagcctacatgcagctgtccagcctgaccagcgaggacagcgccgtgtactactgcgccagaagcacctactacggcggcgactggtacttcaacgtgtggggagccggcaccaccgtgacagtgtctgctgcttcgaccaagggcccatcggtgttccctctggccccttgcagcagaagcaccagcgaatctacagccgccctgggctgcctcgtgaaggactactttcccgagcccgtgaccgtgtcctggaactctggcgctctgacaagcggcgtgcacacctttccagccgtgctccagagcagcggcctgtactctctgagcagcgtcgtgacagtgcccagcagcagcctgggcaccaagacctacacctgtaacgtggaccacaagcccagcaacaccaaggtggacaagcgggtggaatctaagtacggccctccctgccctccttgcccagcccctgaatttctgggcggaccctccgtgttcctgttccccccaaagcccaaggacaccctgatgatcagccggacccccgaagtgacctgcgtggtggtggatgtgtcccaggaagatcccgaggtgcagttcaattggtacgtggacggcgtggaagtgcacaacgccaagaccaagcccagagaggaacagttcaacagcacctaccgggtggtgtccgtgctgaccgtgctgcaccaggactggctgaacggcaaagagtacaagtgcaaggtgtccaacaagggcctgcccagctccatcgagaaaaccatcagcaaggccaagggccagccccgcgagcctcaagtgtataccctgcccccttgccaggaagagatgaccaagaaccaggtgtccctgtggtgtctcgtgaaaggcttctaccccagcgacattgccgtggaatgggagagcaacggccagcccgagaacaactacaagaccaccccccctgtgctggacagcgacggctcattcttcctgtactccaagctgaccgtggacaagagccggtggcaggaaggcaacgtgttcagctgctccgtgatgcacgaggccctgcacaaccactacacccagaagtccctgtctctgtccctgggcaag

SEQ ID NO: 117 - DNA, 639 bp, Artificial Sequence
  Synthetic Construct
cagatcgtgctgagccagagccctgccatcctgagcgcttccccaggcgagaaagtgaccatgacctgcagagccagcagcagcgtgtcctacatccactggttccagcagaagcccggcagcagccccaagccttggatctacgccaccagcaatctggccagcggagtgcctgtgcggtttagcggctctggcagcggcacaagctacagcctgaccatcagccgggtggaagccgaagatgccgccacctactactgccagcagtggaccagcaacccccccacatttggcggaggcaccaagctggaaatcaagcgtacggtggccgctcccagcgtgttcatcttcccacctagcgacgagcagctgaagtccggcacagcctctgtcgtgtgcctgctgaacaacttctacccccgcgaggccaaagtgcagtggaaggtggacaacgccctgcagagcggcaacagccaggaaagcgtgaccgagcaggacagcaaggactccacctacagcctgagcagcaccctgacactgagcaaggccgactacgagaagcacaaggtgtacgcctgcgaagtgacccaccagggcctgtctagccccgtgaccaagagcttcaaccggggcgagtgt

SEQ ID NO: 118 - DNA, 1713 bp, Artificial Sequence; identical to SEQ ID NO: 11
  Synthetic Construct

SEQ ID NO: 119 - DNA, 1026 bp, Artificial Sequence; identical to SEQ ID NO: 12
  Synthetic Construct

SEQ ID NO: 120 - protein, 8 aa, Artificial Sequence
  Synthetic Construct
GYTFTSYN

SEQ ID NO: 121 - protein, 8 aa, Artificial Sequence
  Synthetic Construct
IYPGNGDT

SEQ ID NO: 122 - protein, 14 aa, Artificial Sequence
  Synthetic Construct
ARSTYYGGDWYFNV

SEQ ID NO: 123 - protein, 5 aa, Artificial Sequence
  Synthetic Construct
SSVSY

SEQ ID NO: 124 - protein, 3 aa, Artificial Sequence
  Synthetic Construct
ATS

SEQ ID NO: 125 - protein, 7 aa, Artificial Sequence
  Synthetic Construct
QQWTSNP

SEQ ID NO: 126 - protein, 10 aa, Artificial Sequence
  Synthetic Construct
GYIFTNYNIH

SEQ ID NO: 127 - protein, 10 aa, Artificial Sequence
  Synthetic Construct
AIYPGNGDAP

SEQ ID NO: 128 - protein, 9 aa, Artificial Sequence
  Synthetic Construct
ANWDVAFAY

SEQ ID NO: 129 - protein, 10 aa, Artificial Sequence
  Synthetic Construct
GFTFDDYAMH

SEQ ID NO: 130 - protein, 10 aa, Artificial Sequence
  Synthetic Construct
AITWNSGHID

SEQ ID NO: 131 - protein, 12 aa, Artificial Sequence
  Synthetic Construct
VSYLSTASSLDY

SEQ ID NO: 132 - protein, 10 aa, Artificial Sequence
  Synthetic Construct
GYSFTSYWIH

SEQ ID NO: 133 - protein, 9 aa, Artificial Sequence
  Synthetic Construct
MIDPSDGET

SEQ ID NO: 134 - protein, 14 aa, Artificial Sequence
  Synthetic Construct
LKEYGNYDSFYFDV

SEQ ID NO: 135 - protein, 10 aa, Artificial Sequence
  Synthetic Construct
GFSLTDSSIN

SEQ ID NO: 136 - protein, 9 aa, Artificial Sequence
  Synthetic Construct
MIWGDGRID

SEQ ID NO: 137 - protein, 10 aa, Artificial Sequence
  Synthetic Construct
DGYFPYAMDF

SEQ ID NO: 138 - protein, 11 aa, Artificial Sequence
  Synthetic Construct
KASQDIDRYMA

SEQ ID NO: 139 - protein, 7 aa, Artificial Sequence
  Synthetic Construct
DTSTLQS

SEQ ID NO: 140 - protein, 8 aa, Artificial Sequence
  Synthetic Construct
LQYDNLWT

SEQ ID NO: 141 - protein, 11 aa, Artificial Sequence
  Synthetic Construct
RASQGIRNYLA

SEQ ID NO: 142 - protein, 9 aa, Artificial Sequence
  Synthetic Construct
QRYNRAPYT

SEQ ID NO: 143 - protein, 11 aa, Artificial Sequence
  Synthetic Construct
HASQNIDVWLS

SEQ ID NO: 144 - protein, 9 aa, Artificial Sequence
  Synthetic Construct
QQAHSYPFT

SEQ ID NO: 145 - protein, 15 aa, Artificial Sequence
  Synthetic Construct
RASESVDSYGQSYMH

SEQ ID NO: 146 - protein, 7 aa, Artificial Sequence
  Synthetic Construct
LASNLES

SEQ ID NO: 147 - protein, 9 aa, Artificial Sequence
  Synthetic Construct
QQNAEDSRT

SEQ ID NO: 148 - protein, 10 aa, Artificial Sequence
  Synthetic Construct
GGSGSSGSGG

SEQ ID NO: 149 - protein, 11 aa, Artificial Sequence
  Synthetic Construct
QSLVHNNGNTY

SEQ ID NO: 150 - protein, 120 aa, Artificial Sequence [sequence omitted]

SEQ ID NO: 151 - protein, 107 aa, Artificial Sequence [sequence omitted]

SEQ ID NO: 152 - protein, 121 aa, Artificial Sequence
  Synthetic Construct
QVQLVESGGGVVQPGRSLRLSCAASGFTFTKAWMHWVRQAPGKQLEWVAQIKDKSNSYATYYADSVKGRFTISRDDSKNTLYLQMNSLRAEDTAVYYCRGVYYALSPFDYWGQGTLVTVSS

SEQ ID NO: 153 - protein, 112 aa, Artificial Sequence
  Synthetic Construct
DIVMTQTPLSLSVTPGQPASISCKSSQSLVHNNANTYLSWYLQKPGQSPQSLIYKVSNRFSGVPDRFSGSGSGTDFTLKISRVEAEDVGVYYCGQGTQYPFTFGSGTKVEIK

SEQ ID NO: 154 - protein, 121 aa, Artificial Sequence
  Synthetic Construct
QVQLVESGGGVVQPGRSLRLSCAASGFTFTKAWMHWVRQAPGKGLEWVAQIKDKSNSYATYYADSVKGRFTISRDNSKNTLYLQMNSLRAEDTAVYYCRGVYYALSPFDYWGQGTLVTVSS

SEQ ID NO: 155 - protein, 112 aa, Artificial Sequence
  Synthetic Construct
DIVMTQTPLSLSVTPGQPASISCKSSQSLVHNNGNTYLSWYLQKPGQSPQLLIYKVSNRFSGVPDRFSGSGSGTDFTLKISRVEAEDVGVYYCGQGTQYPFTFGGGTKVEIK

SEQ ID NO: 156 - protein, 124 aa, Artificial Sequence
  Synthetic Construct
QVQLVQSGAEVKKPGSSVKVSCKASGYAFSSYWMNWVRQAPGQGLEWIGQIWPGDGDTNYNQKFKGRATLTADESTSTAYMELSSLRSEDTAVYYCARRETTTVGRYYYAMDYWGQGTTVTVSS

SEQ ID NO: 157 - protein, 111 aa, Artificial Sequence
  Synthetic Construct
DLVLTQSPASLAVSPGQRATITCKASQSVDYDGDSYLNWYQQKPGQPPKLLIYDASNLVSGVPARFSGSGSGTDFTLTINPVEANDTANYYCQQSTEDPWTFGQGTKLEIK

SEQ ID NO: 158 - protein, 121 aa, Artificial Sequence [sequence omitted]

SEQ ID NO: 159 - protein, 106 aa, Artificial Sequence [sequence omitted]

SEQ ID NO: 160 - protein, 120 aa, Artificial Sequence
  Synthetic Construct
QVQLVQSGAEVVKPGASVKVSCKASGYTFTSYYIHWVRQAPGQGLEWIGSIYPGNVNTNYAQKFQGRATLTVDTSISTAYMELSRLRSDDTAVYYCTRSHYGLDWNFDVWGKGTTVTVSS

SEQ ID NO: 161 - protein, 107 aa, Artificial Sequence
  Synthetic Construct
DIQMTQSPSSLSASVGDRVTITCQASQNIYVWLNWYQQKPGKAPKLLIYKASNLHTGVPSRFSGSGSGTDFTLTISSLQPEDIATYYCQQGQTYPYTFGQGTKLEIK

SEQ ID NO: 162 - protein, 120 aa, Artificial Sequence
  Synthetic Construct
QVQLQESGPGLVKPSQTLSLTCTVSGFSLSDYGVHWVRQPPGKGLEWLGVIWAGGGTNYNPSLKSRKTISKDTSKNQVSLKLSSVTAADTAVYYCARDKGYSYYYSMDYWGQGTTVTVSS

SEQ ID NO: 163 - protein, 111 aa, Artificial Sequence
  Synthetic Construct
DIVLTQSPASLAVSPGQRATITCRASESVEYYVTSLMQWYQQKPGQPPKLLIFAASNVESGVPARFSGSGSGTDFTLTINPVEANDVANYYCQQSRKVPYTFGQGTKLEIK

SEQ ID NO: 164 - protein, 120 aa, Artificial Sequence [sequence omitted]

SEQ ID NO: 165 - protein, 107 aa, Artificial Sequence [sequence omitted]

SEQ ID NO: 166 - protein, 118 aa, Artificial Sequence
  Synthetic Construct
QVQLVQSGAEVKKPGSSVKVSCKASGYIFTNYNIHWVKKSPGQGLEWIGAIYPGNGDAPYSQKFQGKATLTADTSTSTTYMELSSLRSEDTAVYYCVRANWDVAFAYWGQGTLVTVSS

SEQ ID NO: 167 - protein, 106 aa, Artificial Sequence
  Synthetic Construct
DIQMTQSPSSLSASVGDRVTITCKASQDIDRYMAWYQDKPGKAPRLLIHDTSTLQSGVPSRFSGSGSGRDYTLTISNLEPEDFATYYCLQYDNLWTFGGGTKVEIK

SEQ ID NO: 168 - protein, 121 aa, Artificial Sequence [sequence omitted]

SEQ ID NO: 169 - protein, 107 aa, Artificial Sequence [sequence omitted]

SEQ ID NO: 170 - protein, 123 aa, Artificial Sequence
  Synthetic Construct
QVQLQQSGPELVKPGASVKISCKASGYSFTSYWIHWIKQRPGQGLEWIGMIDPSDGETRLNQRFQGRATLTVDESTSTAYMQLRSPTSEDSAVYYCTRLKEYGNYDSFYFDVWGAGTLVTVSS

SEQ ID NO: 171 - protein, 107 aa, Artificial Sequence
  Synthetic Construct
DIQMTQSPASLSVSVGDTITLTCHASQNIDVWLSWFQQKPGNIPKLLIYKASNLHTGVPSRFSGSGSGTGFTLTISSLQPEDIATYYCQQAHSYPFTFGGGTKLEIK

SEQ ID NO: 172 - protein, 118 aa, Artificial Sequence
  Synthetic Construct
EVQLKESGPGLVAPGGSLSITCTVSGFSLTDSSINWVRQPPGKGLEWLGMIWGDGRIDYADALKSRLSISKDSSKSQVFLEMTSLRTDDTATYYCARDGYFPYAMDFWGQGTSVTVSS

SEQ ID NO: 173 - protein, 111 aa, Artificial Sequence
  Synthetic Construct
DIVLTQSPASLAVSLGQRATISCRASESVDSYGQSYMHWYQQKAGQPPKLLIYLASNLESGVPARFSGSGSRTDFTLTIDPVQAEDAATYYCQQNAEDSRTFGGGTKLEIK

SEQ ID NO: 174 - protein, 5 aa, Artificial Sequence
  Synthetic Construct
  VARIANT (1)...(5): Can be absent or present, or present in repeats of up to 5 times
GGGGS

SEQ ID NO: 175 - protein, 7 aa, Artificial Sequence
  Synthetic Construct
GQPKAAP

SEQ ID NO: 176 - protein, 5 aa, Artificial Sequence
  Synthetic Construct
DKTHT

SEQ ID NO: 177 - protein, 6 aa, Artificial Sequence
  Synthetic Construct
TKGPSR

SEQ ID NO: 178 - protein, 7 aa, Artificial Sequence
  Synthetic Construct
AASTLQS

SEQ ID NO: 179 - protein, 7 aa, Artificial Sequence
  Synthetic Construct
KASNLHT